European Patent Specification EP 3 722 429 B1, published October 16, 2024. Title: A method for transformation of Gram-positive bacteria. Applicant: Kobe University. The sequence listing filed with the application follows.

SEQUENCE LISTING (35 sequences)

SEQ ID NO: 1 - DNA, 37 bp, Artificial Sequence
  Primer etc.
gagtcagaaaacagacgcataaacgctaacggtcagc

SEQ ID NO: 2 - DNA, 46 bp, Artificial Sequence
  Primer etc.
ctaataccgttccccgagaagcttcactaaattaaagtaataaagc

SEQ ID NO: 3 - DNA, 19 bp, Artificial Sequence
  Primer etc.
agagcgtaagaaacgcatc

SEQ ID NO: 4 - DNA, 19 bp, Artificial Sequence
  Primer etc.
tgcgtctgttttctgactc

SEQ ID NO: 5 - DNA, 18 bp, Artificial Sequence
  Primer
ctcggggaacggtattag

SEQ ID NO: 6 - DNA, 20 bp, Artificial Sequence
  Primer
cgaagatctgcctactgaac

SEQ ID NO: 7 - DNA, 25 bp, Artificial Sequence
  Primer
taaataacatgactgtggaaatgac

SEQ ID NO: 8 - DNA, 44 bp, Artificial Sequence
  Primer
gcttgagtcaattccgctgtcgttagtcttcgatgacgagattg

SEQ ID NO: 9 - DNA, 77 bp, Artificial Sequence
  Primer
ctgattgggtaggatccccgagaaagagcaatctcgtcatcgaagactaaaaaaagaaacacttatttgaacagatc

SEQ ID NO: 10 - DNA, 19 bp, Artificial Sequence
  Primer
gcgtcttcttaaaacgctg

SEQ ID NO: 11 - DNA, 22 bp, Artificial Sequence
  Primer
cgacagcggaattgactcaagc

SEQ ID NO: 12 - DNA, 20 bp, Artificial Sequence
  Primer
cggggatcctacccaatcag

SEQ ID NO: 13 - DNA, 33 bp, Artificial Sequence
  Primer
aaagagcaatctcgtcatcgaagactaaatttc

SEQ ID NO: 14 - DNA, 29 bp, Artificial Sequence
  Primer
ttgttaacgctccttttcatcgatttctg

SEQ ID NO: 15 - DNA, 52 bp, Artificial Sequence
  Primer
cagaaatcgatgaaaaggagcgttaacaagagtgtgttgatagtgcagtatc

SEQ ID NO: 16 - DNA, 56 bp, Artificial Sequence
  Primer
gaaatttagtcttcgatgacgagattgctctttgagtgtgttgatagtgcagtatc

SEQ ID NO: 17 - DNA, 26 bp, Artificial Sequence
  Primer
ctacattccctttagtaacgtgtaac

SEQ ID NO: 18 - DNA, 22 bp, Artificial Sequence
  Primer
gatcgtgaaaggccccaatgtg

SEQ ID NO: 19 - DNA, 61 bp, Artificial Sequence
  Primer
gaaatttagtcttcgatgacgagattgctctttgaagcaaaggattgaaaatgaaaaagcg

SEQ ID NO: 20 - DNA, 57 bp, Artificial Sequence
  Primer
cagaaatcgatgaaaaggagcgttaacaagaagcaaaggattgaaaatgaaaaagcg

SEQ ID NO: 21 - DNA, 57 bp, Artificial Sequence
  Primer
gttacacgttactaaagggaatgtagcactatttttttcatttgcatcactccaaac

SEQ ID NO: 22 - DNA, 26 bp, Artificial Sequence
  Primer
atcagcgaaagcacaaacacaaaacc

SEQ ID NO: 23 - DNA, 28 bp, Artificial Sequence
  Primer
atgataaaatgaccaccgaagaattccg

SEQ ID NO: 24 - DNA, 58 bp, Artificial Sequence
  Primer
gaaatttagtcttcgatgacgagattgctctttcactttcatgtgaatccctcctgcc

SEQ ID NO: 25 - DNA, 55 bp, Artificial Sequence
  Primer
gttacacgttactaaagggaatgtaggaaactatgacagtactgacactcagggc

SEQ ID NO: 26 - DNA, 22 bp, Artificial Sequence
  Primer
gacgagctcaacctttggcagc

SEQ ID NO: 27 - DNA, 23 bp, Artificial Sequence
  Primer
gccaaatggaggccgtatgtcag

SEQ ID NO: 28 - DNA, 64 bp, Artificial Sequence
  Primer
gaaatttagtcttcgatgacgagattgctcttttgaccatttttcagcctcctttttctttttc

SEQ ID NO: 29 - DNA, 61 bp, Artificial Sequence
  Primer
gttacacgttactaaagggaatgtaggattgtaaaagcaaaaagggtgtttcaataaaagg

SEQ ID NO: 30 - DNA, 31 bp, Artificial Sequence
  Primer
ggcttgggatcgatacaagttctttaatgag

SEQ ID NO: 31 - DNA, 26 bp, Artificial Sequence
  Primer
ttcggggacgaaaaatagcacagatc

SEQ ID NO: 32 - DNA, 58 bp, Artificial Sequence
  Primer
gaaatttagtcttcgatgacgagattgctctttctgctgatatgaaaaacctttgccg

SEQ ID NO: 33 - DNA, 50 bp, Artificial Sequence
  Primer
gttacacgttactaaagggaatgtagagccctctgcctttttggttcatg

SEQ ID NO: 34 - DNA, 35 bp, Artificial Sequence
  Primer
gctttgttagtcttcttttgaaagtcagaaaaagc

SEQ ID NO: 35 - DNA, 65512 bp, Bacillus subtilis
tgtgttttaaaatgtttgatgatgccgataagtattaggactagttttgtttttgaatagctggagggaagtgtatgttgtccaaagtaaaaaaagtaccgtctccctatgtaggcaatctgttgaataaatggcatgactatattatgcaggagaaggttcatgagtctatagagaaaagaactgaaataaagcaattgttaagtcaggctgaagataataaggacctggttgattattttattctactggatcatcgtcatagcctttgttttgatcaagaggcatctatgggtgatgtcgttaatatgttaagtaagggaagtcatgatcttttaataaatttttattttgaattgtttgcaggggattatgagttttttaaaaaaaattatgttaaagcaatttctttttatgaaaaagctgaacaaaagttatcgagtattcccaatattgaggaaacgaagtttgcggagtttcactataagattggagttgcttattatgagattgaccagcatttggtgtcagtcaacaaagtaactaaagccagggatatttataaaaaaagtgatatgtggaacctcgaagctattcagtgcagtttggtggtcggtattaatttgtatgatatggggcgtttagatgatgcggatgcatattttcgtgatgccttgactgaggccttggatcatggctatgataagcctataactaagatttaccacaatcttggattagtccattggcaaaaaggttctcttgaattagctctgcattattttagggaagcttattcgcatgaatggttgagggattcgcctaaaggacagcaaactgtatacatgctttcaagagtactgtatacaatggggcaaaatgaagaagcttatcactggtatgaattagggatagaaatggcgcgtaaatttgatgatcatgagtataaagcaaaacacgacattctttatcatctttatgagcagccttcaatcgatgaagtaaagcaatctttagctttcttagaagagcgtaatctttggccggacgtatccaaaattgcaaaaggtatttcagagctttatgaaaaaaaaggtgatttagtgactagtcacgaatttttgaaaagagctttttatgctaaagagcaaattcaaagaataacggaggcgttaggatgaagaaaattaatggttggattgtcgttgctttgcttgctgttactactgtaggagctgcagcagctatacaatacactaataatgctgattctcctggacaatttcaagtagcccaaaaagggatgtattaaaagctgaccaataagtgtcagctttttttgtgttcgatcacggctgcagctgaggagaagatccggcctgaatccggaacccaggaagccaggcgcctatgttcgacagctgaagaaagagatcgataagctattgatcggtaatcagtaaaaaaaggactgcacttaggctagtccttttttaatttcatgtattcatttctaatttttaataattctatctcttctttaacgcgctctatatccttttctgaaagcccagtaacatcaaaaaaacgaataacactattattttcacttgattttaactggtcaatttgattttgaatttgattgatacttgcctcagttaatccagttaaatcaaataattttatctgttttgaagtatctttatctttctctttaacatgatcttcttccattgatgctatatactccattatttgaagcatttctatattaggaatggagagcgccgttgccaactttttaataactgcctgtgtcggtctttttctttcacctttttcaagcatggaaatataagcagatgataaccctgtatcatttgctacttgtgtttggcttaaccctttttgttttcttttttctaacaagtatttagagagatcaaattgctctctattgcccacttataccacctcgcaaaataaaccctgtatacggtctagcgcttacaatttttcgcgttttttttactcagtgaaaaaaaccggttaaaaatttcactgaaatactttacagttaaaaaaatgtctgttatcttagtgaaagagtcagtgaaaaaaatgcagaataaggttttttgttgttaatctcaaacaatttctgtgtaaaaagaactagaattcaacttttgttttaaccaacgtattcactgttgtctctgaagttttaactaccagttaatttaaccgtatgtatgtgtattaatcatacactatcaaagtgtgctatcacaatgtagtcagttaataataagtttagtaaaaacaggataagggccatcaaaatcatgctgcaacttggttttgatatagctcacagtgaaagttagtgtgaacttgccccatttattgtattcatacatcattttagctttaaaagagaggcatcttttgaagtaaaattcatttggatgtatgtttatcaatttggagctgtcagactaactgacagctttttttgttgtctttacactgattgaaaatttagggagggaatagcttggctaaagttaaattgctcgaaaaaaaaatgactgaaaaagatgttttagagtatggaagctctttaagattgtttgacggcagcactcatgtgttgatcggtaaggattgtttacatactcatacaaaaaataaaagaccgatttcacaatgttattcggatattcgaaacgtgaagaacgttgagggtgttattgtgggaaaacgggtttctccgcattctagtcttctttttacgactgaagcctttcagccggcaagaaaagtaacccaggtatataaagctccaaaaatgccgcgtagaagtacacaagtacggccgagaaatacctctggaagagctaagaaggtatcagttcttttaagtgaaactggatatgcaaatgttcatcagctgaaacaagtgttacttgatgctggtgctaaaaaagtccaaacatataacacaagcagaggcattgctatcgtttgtcatcctaatcctaactatttgctacaaaaagtaatttctgaataaagtgaggttgatcaggattcacacgtttatcagtgattaagctgataaagaattaaatattagggaaggtccccctccaaaggtataacggccatgcaatacctttgggtgaacatttcttcttggcgcgagtgacggttttcaccggtcgtagacggcaagtttggccttacattatcagattcagatgaagttaagtctgaatacttggctgatatagagttccgtgagtaacaactgctacaaactcacgattttggactgtttcattgataaacgtgtgaatcctggcttccaagtcaaattacatcatatgtttttaactcaaaccatagtaaaattgtgaatggaaaaatatatttaaaaaggtgttgagtgtaagtatgagaaagaaattggctgctggtattgttgccggtgcaattattttaggagtgcctggctatacaatttttcattcataccaagcaaatgctgaagaagctcgtgtgttagacaatgcaacggatgcagttaactcattatatgcttctaaaaaatataattacttggctgatggggtttcaaagaatgatattcaaaaggctcagaagttagtatccgatgtagctgattctaagaaacagaaatcattagcagaaaaagcatctaatgctgcgatcatgttagaggcctcaaatgcagttaaagaggatatcgttgacggggtgatcgttgatgatctcacaaagtctattctttctgttaccaaggaaagcgtagataaggtaaagccgatcagcaaagatttgtataaagatttatctaaagacttatctaaagcttatgatcaaattgaacaaatagacaaaacaaaaaaattactcaaagatgcgaagaaagattggaattcctataaaaagattgaaaaagaagtaaataagatttccaatcagactgcgaaaaagagtctgaaaaaacagcttgaaacgctaaaaaagagaattgaagatcaagagtctataagcaaaaaagcgaaagaaaagctgaatgagattgagaaaacgtcacagaaggacagtgacagtaaagcagcaaacgacagcagtcaagtaagcacaaacgataatgaaaatgctacttcaagtgcggcatcaagtaatacttctgcaacacagaataaatcaggtagctcgtccaattcaagcagcagttcgggatcatcgaattccgggtacagctcatattcaaacgggtctagtaaatcaagctccaacacgaaatcatactcaaattcttcttcatcaagatcctatacatctaagtcaaattcgggcagcactagccatagcgaaagtaaaaaaagcagaactggaagcagttcagctgggagcagcaataaatcatcaagcagtaagtcgtcttccagcacatctaaaagtaaacaatcccaaaacaacaccatgaaaaatgcgaacgattttgttaatgactttaacagtggaaattataatcatgttggtagtggtaataatgggacaggtaataactacgatgtgtatgagagaggacagtaagcattgggtgataacacgaataaatacgtggtctctctgatttcggtattcattgctggtttaatagtgttaattggtcttatggcgttaagtggggtgtatgcacagattgaggaaaggcagtctgaaaaaagatatcaggcagtttcaactcaattaggcattccaaaagctgagatcctaataacaccttctgcccatgacggaatctatactgtaaaagctaacaacaggttatacttagtagagtttgacacctcagataaaaaaattgcacatatgactgaagaacggactaattgattagtccgttctttacgttttttaataaagaaaaaggggcttgtggaatgaaaaagattttgctaattctaacatttgtaatcctggcattttcagctttaaccggctgtagcagtgagagctgggatcgcacagtaaaagatcatgaatcaagtgttaacgggctgaaacgcacagcaacggtatatgaccaaaatgggaaggtcatcaagacgtataaaggcaagtttgatgtagaggtcaatgattacggaaataaagttaagtttgacattgatggtaagcgcgtggttatcaataacgcgatagtgattgtagaagaggataaatgatcgaatagcaaaggggaggtgatgatgaatgttcctattttgaggtgaaaggagatagccatggatgaaaaagctattttaagtgatgaagtggccaaggataggatattaaaccgaatttccagtgaagggattagaataagatcttccttttctaagtctgcgactgggcaatatacgtattatttgggagaagataagataccgccgacaattgaagtaccacaattcactgatctcagtgaattaatacaggcatttgcgttggcgcatgaattgggacatcattacgtataccaaaggatttcaagaaaaaaagctcggcttttcaaatctggaatgacttgtacaacgtattggaatgagaaattggcatggcgggaagccgaaaaaatactgaaggaggaagggattctagttgacgagcagaccaactgctctttctttaagtacaagacattttgcttaaacacttataaagatcaggtggtacattctattagcagcccgttcaagttcttgttcggcagtgttctgcttctaatgtagctatacatcggactttatattctacttggtattgggctggttttttccgcgaattctatcccaataccatttgatgaatttttagggttcagttctttaaataaaaatgaactccttactgtcgttcctaaacttgtttacatcttgttaagtttagccactatgtataagttttgttggtgttactttttaaagcgctcatttagaccggctctattttattttgtaacattgtttctctcacaattggcccctatggtgctctagagagaaaaatggatttggaaaatgaggtggaaaaatggatttgaataaaggtattgaagaactgcaatctgaaaatagtctcaaaggggtactattagagggacgcctagaattcaaaaagtttcttaaaaaaaataaccatttagatattaaggatatccactggcaagcaatacaacataattcgtggatagaacactatttttttgttaagtacaccgagaagaatggtgaattaaaggtataggaggaatctttgttgaggcaaatcattatacttcccccatcgggatttgtttctttgagtttgtttaagcttttgccatacagcacaataagaaaggggtgatcgaagtgattcacatagtgtataaaagaatcttgataatgctatcaagtgttgtagcaattgccgcagcgctttttttagtgccatttttcacctcatcggccgaagctgctacagctgttgccacaggtccgtattcatggaaagatccgcacggcattactcatgaatcagcttacatcaaaataggagacaccattgtttactgtattgatccagataagcctgcaccttatggcggtcattcgtataaaaccccgaagcgtcaatatgatgatggcgtcaaagccattctttattacgggttcggcggtgacggtaatgaaattggaaagacaatgacggatatggtcaaaacctatgtcgctcttaacaactggctagatggaaaaagggatcaaagaacatatagtaaccaggatgccgaagtgtggaagttaattcaacatgctaaaaaaggtgatgctccgagctaccaggtatccttcagcaaaactaaagtaggcagctctgtttccggtgatcagcaaaaatcagaaaccattaagctgaacgggaaaggaacagctacgttaaccgttccttcaaaggtaacgatacacgtgatcggcggcaaaacccaaaagggcggccatatcactattcatgatggccaatcattttatttcactgcacctttagattatggatctgactacgacacagggaatgttaatggtgagatcagacagctggcgtccctgctttatctacctaatacgagcagctatcaacggctgatgtcaagtacatttgtggttgatccggttgtggcagctggttttaccgttcattttgaaaagcgtcaaaaacaaattacggtggttcataaggacaagtacgaaggcacggtcttaaagaaagtaaaagagtctaaaaatatcggaaccaattacagctattcacctgagaagaaaatcgtaaaagatgggaaaacctatgtgcccgttaaaacagaaaagaaaaccggtaaattgggaaacaaagatatcactattacttttgagtatgcattgcaaaggaaaataactgtgctgcacaaagataaccgggaccacacgttgatcaagaaacaagtatataccaaaaaacgaggcgatacgtattcgtatggtccattaaccaatttgaaaaagaacaattacacatatcgtcctgtctcggataaaaaggtaactggtaccgttggaaaagatgatgtaacaattactatttattatgatgttccattgatcaagaccagccttgataagcttcaaatatatacggctccggctgctgatggtctgccggttaaggtttatctttctaagaccaacatttataaaaatgacaccaagggcatgaccacagcaaaaataaatgtcagcttgtatgacgggaaacagctgctaagcaaaaaaacatatacagcacagagtttgccgaagaatgtaaatttcactgtgccggcaaagaatttaaaggttaacgcaaataaactctatacggtcaaattagagggttttaatgaaaatgatgtagatgtacctgacaaggcaaaagaactctctacgaagggttatacgagttctgaagacaaagtttctgtgtctatgaaagttgtagttaaaaatcagggatctgttaaacgcgtagttatgacagaagtaaccccaacaactgctatgaaaagctattttgaaacaatgacatatcaagggcagctgcttcctaaacggaaaaccggttatggcagcgagcaaaatcttgctttcatatatgagaacatgcttcaaaaagacgatgatgatatcaaattcgattttaaagtacctgaagagttgatggatacttacttaaactattctgttaaagacggtaaagctatattccctatggatgttgcagcatctaagaaatcaagcaccgcagacaatttaatccgggaaatgtcatttgttttccctcacgtaaatgtggaaaaagaaactggcagcttattcacagatcagcaagttaaagcaaaagacaaacgcttgaaaaacgctgttcgtgacggagggaacaaattttacactcctatttgggcggaattaggcagctatgatgtttcttatacttcaagcaaagtaggggttaacaaagtgactattgaattgaaggataagctcacactatttgcttatatgtacggccatatgaattcagaaacaaaggatcaggacgaaataatgctaacgccgattaatgctgatgatcctttccctaacggtacacctgacggctggtcacaaagtgatattaattggttgaagaaataaccttttcaactgtttggaggaaaaagtatggagaaaagctgtttcacttttaccaccaagaatagggttgaggccatcacaaaaataacgagactcatatctgaaggcaaattaatcagcgttaattctagaagaattaaagaatccacaaaaaggcagagccttcagccgatagacgatttatatacaggcactattgagtacacgattgtcagctacaaagaatagcagcagagcaatcagaaagggaaggtaatgggttatcaagataaaggaatagacgtacgttttctaatatttctactcaatgtaggttatattgtacttggtatagacagtgtgcaatattactctaaagcgagtttgattatgttctgtgttctcgtagcctgtaatttaagcatgctgtttttttatggtgtataccttagagaacaaagacgggatgatctttgtattgtgaaaaaagagctaagtagacatttaaaaaaagatgtagatgaaattgaatttgagaaccatcacaaaattggacatagattgtatggtatagaagcagacggcgttttatatcgcgttttagtaaaggaaaaagccgagatagttaaagggaactaacttttagttccctttttttgatacctggagaaaatcgaggtgagaaaatgaaaggttcgattaccactttaggacttgtatatattggcctgtttctgctgatggtcatcatttcttatcacaccgaggcataccgacacaattcgattataagcactatgaccgaatcaggacagatagcaagtatcaacagcattgataaaagttcccgtgtggaagatggacgtgtagaggttacagaagagagcttcaaaaagaaattcaaaactctctttgaacaaaacagcaatattaaactatcaggaactaaatataactttgattttttaaagacagcagacggcggaattaaggctgtccgcgttaaaatcacagacgaccgcaactcaaaatatcaagtaacgttcgtgtcgaattttgtcagttgaggaggaaataaaatgattagtccagatacaattaaaggtatatatacagatatccgagagaaaaacccagaaattgtgttagaagctttcacttcaaaagaagcaagggaagttatgtggaaactggttgctgaagataatgctactgttttggatactgataaaaaagtagattatgtaatgcaggaaatggttggcctgggtgtcattgaaacgattataaaacaacatgatacggttacagatattacttttaatgcaaatcaattgattgttagaagaagcgatctcaaagacccttatccatacgaagatcaggaaataactgaggagtatattttaaagatcatccaaaagttcgctaatgcagtagaaaaagaatttacacctaaagatcctatcttggatgcctctttggggaatttgcgaatcaacgctgttcataaagctgtatcgccatatgggaccacaatggcaattcgcgtatcacgtccaaagctggcacttaccaaggagaatttttcagactttgctcctgactatatgtatgaattttttaaggctgctgttgcagcaaaagctaacattggtatttctggtgaaacaggttccggtaaaaccgaatttcaaaagtttttgttaagctttataccatttggagaaaaaatcatttggattgaagatacgcgggaaggacaccttaaagagttgtttggggacacaaaagatattcatagctggcttacttctcctggggtaactattacagatttggtaaaggcggcactcagaaacaaccctaaatggatctgcgtatctgagacgagaggtatggaagcatatgaaatgctgcaagctgttttgtccagtcacagtatcataaccactttgcatgcaaatgatgttaagactattcctcgaagatttatcaatatgatgaaaatgggctaccaattagatgaaaaatcaacacttggtgatatttatgaaaacttccatttaggagttcatttgaaagccacagagttgaatggcaaaacggttagatatctgagtgaggtttccgagtacaatgctgatggatctgtaaaaatgatcttcaagcaggagcacatagacgggcgattcgtgcaaacagtaggtaaaataagtcagaaattaaaggaccgcatgttagaacaccacgtcaaatatagtggtttacctgttaggggggaatagtgtgaagaaaaaggtatattcgctagatgagcttaacgcttataaagtcgcgtatggaaagcctattgaacgaaaagagcttttaatgtctttgataaaaccatttgctgtggtttttgttttttcttatgcactgttttattactggtggctcagcttaatattaggtgtgtttgcaatgttttatggctatcgtgttatgatgccgcagtcaattaagcgtgtatacgaggctaatgcttttcaagagcgtcataactttgttaacaacttaactcaaatccttaccaattccgataagactatgttaaaagcattagaaacagtctcggatcgtgcaaaaggagaatttaaagaggatcttcttcagctgcgaggagcgcttcaaggtgcttctactgaagagattcatgcagcatttaaagagtttggtgagaaatataagcatgacgcaatatttgacttgtatatcgaacaattaactactgctactattgagggccgtacaaatattgaaacgattaaagatataaaatcactacacaatgaattgaaacaagaacaagataaatttttacagaaaaagaaacgagctacgtatgaattcaggtttatttctatcatttctttagtattgatcgcggcagtgacattttcatttggctggactcaatgggttaacatttatgctcaccagctgccaggatggatttcaagttcaatttatctcaccttattaggtgtgtttttccgttcttaccttaaaagattgggtgacgacaatttaatggaggtaaaattatgactgctgaaatcattgaatctaaaaacaacaacttttggttgaaatgtgctgaaagtaatttagcttccatgctagatgaaatgggatatacacagcaatgggtaacgagcttccaaaaaaaacgccttatgaaagcaattattgctttagctgttggtgcagtagtaggggcattgtttagtacctggatgatgttattagggcctatactggctgtatttgtatggatgctggaatatcaaagaattgtaaatgcgtacaaaagacatcaatttgaaaaggaacttcaattcaataagtttattagaatgttgtttccgttgttattagagaggaatgctacattatacggtgcattaaataagatgctcaaaagaatggatgatgggcatgtgaaaactgctttaaaacggtttttaatcggattgagcgatgaacctaactcagaagctcctttccgtttatttgctaaagaagctagtgggacggatagagctatgttaatcatggctacgctttttgattaccagcaaagttcaaatgatacaacaattattagtgaactaggtcagatgtcgagtaaacaattatttgaaggggtaagggaaattgctgaatttaaactaagaaaattttatatgttcccaacaaagctcacaatggccagttttgttcccatcgtaggttacgcggctgccatgatgatagatactattgcaaaattatctttataaaacactgaaagaggtgtaagacatgcttgatggagcagtaatggccatagggaaaatgtatatggccattttcattttatttgggattttttctgcttcagctttttttatacagatgaatcagggaaatgaatacaagcaatatattaactatcagattgagagaaacggcggacttacatcttcagcaatggatcatattgaggaatataacaaaaagtattacgaaagccggttcacaattgatagtccgatgatgaatcaaaaagttaagtatggagatgaagttaattacactgtaaaagggaactttaaaattctatattttgacctcccgattcagacggtctcattaaaaggttctgctttatcgttgattcgataatgtagggcctttttatattgcgctcttttaagggggtgagggatatattagatcaaaacgccgacaggatgtattgggtgattggtgcagtcttagtagtaggggctttaataggactttctgtaaaagaatatccggatatattaaacaacgtttttagtggttttacagctaaaataccaaaattttaattcgaatacacaataggagagtgcaaacatgttagatcaaaacgcagacagaatgtattgggtgattggtgcagtgttagtggtaggagccttgattggccttgctgagaaggaattccccggcttattaagcagtgtatttagtggctttacatcgaaacttaaattctaattttagtaaataggagagtgtaaaacatgttagatcaaaacgcagacagaatgtattgggtaattggtgcagtgttagtagtaggggctttgatcggtcttgctgagaaggaattccctggtttgttaagcagcgtattcagtggttttacatcaaaacttaaattctaacggaagagacgtacagctgtatgtttctttttttttgaaaggaggcggatcaaaaatgaataaagatggaccggtcgttaaggtcaaggttacgccaaaacaattgcattccatgatccataaacgccaggcaagactccctcttggttaccaggtgaccaagggggggaagtttgacgcttactgtgatcaaaaaagtttgcttcatcaatttgttatcaaaaacttcactattaaaaacaaccacatcttagtgaaattcactagctgatgatttcatcaattgaaggaggtgaggagaatggctgctacaaaagccgagaaaaaagatgctaaagacctttgtgaattgatattagcgtcacaagggatttcctatgatgattggcttcatgatcaacataatgcagttgtttctaagcacagtaatattttgaagaaagcagtaaaacaaatggtaagtaaaccagcaacttcagagcaacacaactaaaaaatgcaatcaaaataaattataagaggtgtcattcatgccagataatattgtagatatgcttacttacttaattagagctattcaagttgtcgtcggtgcctacgctgctcttaaactaggtatttacgcttatggatttatgtctaaaaaccaacataagactgaagaggcgaagggcggcatgaaaaatgtaatcattggtcttgctgtagtagcaggctgtgagccgattgtaaagtggattcaaaacggtataggtttctaaatgaaagtgggggtatctaaatgattcgagcttcgtttaagggtgggagaaaatttcgatccattattccatccagaaaacaatacagtatacgtttagcttcctcgaaaatggcggaattagagagatttgctgaggaaaataaccttaatgcggaaatagtattaactatctttgacgatgaagataattcagttctctttcgggaatctttttctgttggagaagggatttcgaacaacctactctttctcgtaagcagaacattagatactacttttaaagacagtccgcaggaagaaaaagatgcattgcttcaaatgttatcaaaagccatggaagaggaagctgttgaacaggaatgtaataagaagctgttttcagttccgaatttaggtttttttaaaggcagaaagaaaaatgaactagatcctaaggcagccgaggcagagcgtgcccgccaggctgaagagaaggcccggcaggaggcagccgaggcagagcgtgcccgccaggctgaagagaaggcccggcaggaggcagccgaggcagagcgtgcccgccaggctgaagagaaggcccggcaggaggcagccgaggcagagcgtgcccgccaggctgaagaggaagcccggcaggaggcagctgaggcagagcgtgcccgccaggctgaagagaaggcccggcaggaggcagctgaggcagagcgtgcccgccaggctgaagaggaagcccggcaggaggcagctgaagcagagcgtgcccgccaggctgaagagaaggcccggcaggaggcagccgaggcagagcgtgcccgccaggctgaagagaaggcccggcaggaggcagccgaggcagagcgtgcccgccaggctgaagaggaagcccggcaggaggcagctgaagcagagcgtgcccgccaggctgaagagaaggcccggcaagaggcagctgaggcagagcgtgcccgccaggctgaagaaattgtcgaggaaaacaaaaaaggaaaaccagctgcagctgtaaaaacgcatttatccaatggattcagtaaaggaatagcttttcttaaaaagcagaaacagtatgtacctgatcgtaaaaataaacgtgaaatacatccgcctatagtggcacaagaatcagctgctatgcgtgaccttgaaaagcaacttaagatggccaagattgaattgattgaagaaattaagaaagaaaaactagaattagataaaaagttggctaaagaaaagaaaaaggaagacaaacataagaaagctttggccaaacgtagaaaacgaatggcagcgcctgggcttgggtcctccaagctcattttgtttgccattcttcttattatcggcgtacaggtttatttcaacgttgaatcaggaaatagcccgctaacagttcccggctgggtaattgacattggaaataaggtcagcaacctagtagcctcttacaaaaagctttaacattgttaagcagaaaggaggaagctttggccaataacgttgatcgatatgatgttgatatggaaaagaaggcgtcaccttatctaaatgctcttggatcggctctcagcgaaggcaaaaaaagagctttaaatgaacttaatcaagccaataccttcctgaacaaaatctttaacagaaaaaaaattaatcaattgtccgaaaaggtaaagctttataactactgtgagaaccaagtaagaagtagcgatttcagaagcaagttttctaaaattgagattctagctggaagagaatctcaaataaatattaatgtatttggggaacgaattgaaacagctttaggaagctacttcaaagaacaaggagaaaacttgactcctggaaatagtcttgaagcgtatgatgagttgtataggacaatggttaactcacaaaccttttcatctttacgaggtaataatttcacaggcagatcagaacaagatacaagtttgatgggatttatttcttctcaaaacgagtatcagaattatgtggccgattatcgtgagtctaaaccaattcatcaaatctttccagaccagttcaaggaaggcatgttggagaatgaaagtaaactttacatcaacgagtatacaaaacatttagcgttagttcatgacgagaacagatctatgttgaagaatgaatccccagattacgctgtcatcaaagagttggaaggagaaattcgttctaattttagtaaagatccggaatatccggttattttattaaggacaatggcagcagataaccttaataaacagatagcaactgctgttaatatgactaactcctttattaatgatttttctaaagagatgaaaattaaacaagtaccttggcctacaactgtgcctgaacctctaacttatgagcagtataatcaaaataaatctaaatatcttgaacagctatcaaaagatgatgtgctgatgaaaaaaaatgaaaaagatctgtcaactgaaagggaactagagaataaagggactgaaaaaggaaaagttgaagttcaaattaaaaagccctcaaatttgaaaggttcaagaaaagttaaaggtctagaaagataatagaagtgaggaagccgtgtttacggcttctttttttgaggtgatcttttgcacaaggagtttaaacagtggaaaaaagtatttgcagataagtattttttgattgcctttacactgttttgttatgtagcagtgacgtgtattactaattttttcatacatcttttaaaacagattcccgtaatactctcttcttttaaaaactttgaccagtcacagctttcaagtccttttagttcgatgacctggaagtggttttttgaatttgattggagtatgggcattgtttatggagtagtgtacgttcttgcttcaattttcatattgagacaagtgtataggtttagaatcgcttttcgtgatatcaataagcaaacgaaaggtacagcacgatggactgagattatggagattcaagaaacctataaggctgttaaagatgatgataatgagtatgaaggcagtgcaggaatgccgattgttcattttaatgaccatctttacgttgacacaaactcaactcatacccttgtggttgcttcaacacaatctggtaagactgaaacttattcctatccatatttagatgtcattatgagagcaaaagaaaaagactctgtagtaattacagatataaaaggtgacatgcttaaaaatacccgcgctgaattcgaaaagtacggttatgaagttatgtgtttcaacttattgaatccgtattggggaatggcctataatccattggaattagttaaacaagcatatttgaagaaagactattctaaagcccaaatgctttgtaatacactatcttactcactgttccataatgataagtcacatgcagatcctatgtgggaaaatgcatctattgcattggtaaacgccttgattctcgcggtttgtgatttgtgcattaagaatggacagccagaaaatatcacgatgtatacattgacagttatgttaaacgaacttggaagtaatccagatgaagacgggtatacacgacttgatcatttctttggtaatttgccgccttctcaccctgctaagttacagtatgggacaattcaattttcacaaggcataacacgcagcggtatttacacaggtacaatggccaaacttaaaaactatacttacgatacaatcgcccgaatgacagctcgtaatgacttgaatattgaggatttagcttacggagaaaaaccagtcgcgttattcattgtctaccccgattgggatgattctaactacactattatttctactttcttatcacaagtaaacgctgtgctttccgagaaagctacattatccaaagaaagtacacttccaaggaaagtaaggtttctctttgaagaagtcgctaatatcccgccaattgaagggttaaatagatccctggcagttggtctaagccgaggtatgctctatacgcttgttattcaaaacgtttctcagctacgtgatgtctacggagacgacatggccgtggcaataatggggaacttgggtaaccagatttacattatgagtgacgagtgggaggacgccgaaaagtttagtgaaaaattgggtgttaccacggtaatttctgcagatcgtcagggtgatttaatggacgttcataaatcgtatagcgaaagagaagaagaaaggcctttaatgcttcctgacgagctaagaaggttgaaaaaaggtgagtgggttgttttaaggactaaaaaacgtgaggacttaaaaagaaatagggtagttccttatccgatttttgcttctttagataacggaacaaatatgctgcatagatacgagtatttgatgcatcgttttgataataagattgctcttggtgatttagggtttagaggagagcatgaaacactggatctggaaagcttattgattgaatttgaatttaatgaacctgtgaaggaggaaagaaaaagtaaaccaggtaaagggaaaaaacaaaaagctaaaaaggctcctggtgaacctgtttctagtgaattcccattgcctgaagaaccgattgggtttactgaatcttcagagggaatggattcactattcgcctcaattccagttgagaatatgaacgaacatggattttatgaagatccgccaatgaatgaatcattacatgaagatgatttagaagcaagtgaggaggatattattatgaattcacttgaagaggtgtacgaaacgagtacacctatttctgatgcaattaaacctgatcattacgtgtatataaagttacttgctcataagcaattatctgaaagcgaatatgcgtatttcgatagtctgaaaacagttgaggaattaagggccttttttagagcgccagagaaaaaagaaatttatgaacaaattaaaacacatatagagtaagtgagggttgtttatggatgattcagagattctgaaaatactgcttaggtttcaagattacctatccctgacttcaatttggaccgcaccattccgagtcatcggatggtgggttattatgggcctggccgcaattgtagatgccctatctggggggattgaagagatttatgatttgcttaatttcttcgatagtgaccaaattagtggctttatagataagtggatgcctgtcatttttgcattaatggcattggcgcttggctttcttggatggaaaatcatagttcagaagaaaactgattacgacaaaataatcacaaattcattatttgctttaactcttttccttgtactgccatgggggatgcagcaggcgtcggatctcttgcttgctgggaaaggaatgcttgatgaagacggaaagcttagtgtttccactaaaatatatcaaaacaatatagtcgatgtttataaaatcgacaaggatgctgagtggagtaagaaagaattcaaaaagctaaagaagaaaaataatatcgagaatgacgaggatgtgaaacttttagatataacggagccagttgatacaggtggaatttttcactctagtccgttaactaaagatggcgaaaaaatattagataaaaaagtaagcgatgcatccggagagaagaaattagaggatcttgagtcattttggatacaagatgatgaagcctattatcgatattcttggcacccttggtacatgatgtttgaacttggtaccatagcatttgttttatttatgaccatgtttaagacagcgcagttaatcatggaactaggaatcttaaagattttcagtgtaggaactgctttaacggatcttgaaaacggtcaacgtaataaaaagttcttggagaagataaagaatactttcattgtcttattttcaatcgagcttttgttacaatgttacatcctttttacagattacattggccaagctgacatatctgcaccaataaaaatagttgtattgattgcagcagctattttaacggtggatggtcctaactttatagaagaaatgtttggtatagattctggattgaagagcatttcgcggagtttagttgggctatttgcaggtgctaaaacagcaaaaatggctacggactttacggcatcaacagctaaaaaggcggggaaaatggcaggcaaaattgccaagaaatcatctgatgctgctttagttggtatgggtgctggaaagggtatacttgatggttttaaagagaacatggaagctgctaaaagtggtggaggaagtaacggggggaaaattggaaaagacggtgacacgcctttgtcacatggattagccggtaaaccgactaatgttatgtcagacgatgctttaaaagaagcaatgatgtctggtgacgatcagaaagagaaggataaatcgtcacaatctgattctccgttgtcgtctttgaataaagaaaatagctccgattcatcaacagagggtatcgaaaatcgcgatgatagatcaggcacagaaaatggatctccaatggaagatcataatacaccactatcatccatgtcttccgaagaagaagctggaagcaacaatgagaaaggatcagacaatattctatcaaaagatggagatacaccattacaagcatcaaaagatcagtcgagtcctgatgcagctagtgatggtctaggtactcagcaaggtaaaaacattgaaatggccactgacaaagacggaaatacaccgttgtctaatatggcatcatctgaaggaatacaacctgatcaaccaggtggatctgctgctgacaaagacggagatacaccgttatctaatatggcatcatctgaaggggcacaacctggtcagtcaggtgggactgctgctgacaaagatggaaatacaccgttgtctaacatgacaggggaaagctcagttccaggacaaggcggcggaaacgcgccaggaagctctgatacgccattatcgtcccaagggccaacaggaagtccaattccaggacaaggcggcggaaacgcgtcaggaagctctgatacgccattatcgccccaagggccaacaggaatcccagttccaggacaaggcggcggaaacgcgccaggaagctctgatacgccattatcgtcccaagggccaacaggaatcccagttccaggacaaggcggcggaaacgtaccaggaagctctactaatacgccattgtcatctcaaataccacctgtaggaccaatttctagtcagatcggtggaaacacatcagttacacctggtagacaattgtctcaggggccgattaatagtggtctcacagcaaacaatagcacttccaataatggatgggattcgttgtttgcgactatgccacagaatacaggttcacattcttcaggaagtcttatgccgagcagtcctatttcacaggcggcgccggcttcactgacacctgttgcaccaagcagtaatacatcgatagtaaattccgtttcaaatggttctaattcaacttattcggcgcctacaccggcaagtaacattttgccaacccaccgcgctgccgtaggaaatgttttaccaacctatagagcacctgtacaaaatatgggaggtggccgttttgattactcacctaaaggagtgagtacagtaagcaataaaccgattggaatgcctaaacatgttcaaacaactgcagaagcatttaaaaatcagatgacaaaaaggccaactacgaatatgactgcaaaggatgtcttggttaataagtatgctgacttggcgcaacggatatatgattcaaagtcagtaagaaattcaaggacagcttacgatatcgcaaaaaacactgtaaatactggattcaaaggggggactgataaatgaggcaaaccgtatcagtaccagaaaatattcaagcaaaaatacaatggaataaactaacggttgtggatggttttgtgattattgggagtttggctgtcgggtatttcatgaaaggcttggtatacccgtatcttcagataccttttgtattatttatcgtgcttgccactacattttatctttggccgtgtcctgattcaccaagtaaaaagatttatgaaatgacgctcatggttttcagaaaggatagtcggacatataaagcacaagagcctgtcaattattccatgataaagcaggaggattaaaatgggttttgatgcactgtcagttaaaaagaagaatcaatcaggaagtacacggaaattaaaaaaaatacaaaagagtattgatcgaatcaatcgtgtatatccggtatgtggatatactgatgagggttatgtaaaaacaaaatttggactaaaagaaggctactttgaggtatttgacgttaaacattatgacaccaatatcctagacgaaaaagagtttaactttgtaacagagtcctactggaaactacagcaaatttattcagatcctcttaaagaagtgcatatgaatttgcctgaagataatcagcttcagcaagaatatattaaatacaaaattgaacgaacaaataactttgcaaggttgagagtattaaacgctgaactcgaaaagttgaaattcatagaaaaaacatataaaagtcgtcgcacgtacctcattgtctttggaagaacagcagaagaacttactaaaaggattgacgatttaactcgctttacaaactttttagaaccgcagccgatttctatcgagaaaaaaattaagatcttacatggtatgaataactttatttaggcggtgaatggatatggaaaaaattattaaggatttagattttgtgtatgccacccaaccaatgggtggcatttcttttaaggatgaattttttaatcgtacaggtgatggatatgttgcttgtctccatgtataccgttatccggaaaatttcacaccatactggttaaacaaattaactagtattcataacacaattgttactattgatacctatacacaaaaagacatcaattatactgataaggtaaaaagctcgactaatgaaatgaaatcgaggatacgtaatgcagctaatgaaacagatgcagatgtagctcgtgaagaattgcagactttaagagaactcgggttggctattaccaaaggtggagaagtaattaaacagattcacgtccggatctttttgcatggtgccacacaatcggaattagaaaaacgtatatctgaagttcaaaagagtattgacagtgatggttttaaaagtaaagtgtttcttgatgaaaataaagaagaatggcaatccttatttcttgattatgaaactcaattaaccatgccaaacaaaagaataggaaatgatatgcctgctgaggccattggtttaggttttgcttatgatcaaaccagtctaagtgatccaacaggtgtttattatggttatacatcaacgagaggaacagtttattgggatttgttccataagacaactaaaaggctatattataacatgtttgtggcaggggatatgggatcaggtaagtcaacacttctaaaaaagatcctaagagataatgcttcaaaaggtaactttattcggggctttgataaatcaggtgaatttcaatccgttacggctgatatgggcggaattactattgatttggatgggagcaacggccgtataaatttaatgcagatattcccgtctgtgacaaagaaaataggggacaaagtcgtaatagacgaaagtgcttcttttaggcagcatgtttcaaaattaaattcgtgttaccgaattaaaaaccctaaatccgatgataatgttttagttcaatttgatgaattagtatatggattttacgagaagcataacttttggggagaagatgcacgctccaatatcactcaattacctcctgaagaatatccattattatctgattttcaagcatattgtgaagaaagatatcatgcagaaaaagatccaaatttcaagtccagaattggcgacatagctatgtcaataaagaaccttgttactcaatttggagagatatttgatggtattactactattccggatatggtgaatgaacagatcgtattttacgacatcggaaacctgtcacagctgagcgatcaagtaaaggatatccaaatatttaatgcgctcagtcaaatttggggtacgatgatgaatattggaagaaaagaaaaagaagcttatgataaaggtaaaatacattggttcgatattacgagattccttattatacttgatgagtgtcacaatttgttggaattgaaaaaagctcacaccgcgaacttttttgttactcttatgtctgaagcacgtaagttctttggtggtctggtattggctacacagcgtattgaacggatgtttccgaataccaatacttctgatccagatatggctatagcagcaaataaacttcgtgaaatatttgggttaactcagtataaagctctgttcaaacaagatcagacttcaatgaaattaattaagaatttatttgaagaccaaatgacagacaatgagtatgctctgctgcctaaatttgaaactggtgattgtattctttcgatagctggggatcgtaatttagttatgcatgtagaggctacccaagaggaacttgaactgtttgaaggtggggcttaatgttgaaaaagattccggcaaatgaagaaaatgcagaaaaaaagattgttaggcaaaagaagctgtttatagtcatatgtattgtttttattggggctatgctgctttattttatgggcggaagtaataaagaaaaggtaacaaagaatgaacaaaaagaaagcttaattgaagggaatagttcagagcaatcaacctacaaaagttctgtcgtgaaggaagaaaaagcagaggataaagataaacaagaaatgcaacaaacactgaaatcctttatagaatcatattactcgtacgattataaaaataaagacaaacatttaaaggagtcaaaaaaatatttgactccggagttttataaggaattaagtcttgctgaagaaaacaatacaaaagtgcagcctttcgcttatcgaaaagtacaggacatttcttattcaggcttctctttagtaaacggaaagcctcattggattgccagtgttaatgctgaattattggatgataagaggaaggtcactggcactattgaagttgaatttgaattggatttaaacaaaagagaagataattggaccgtaacatattttgctgtaacaggtaaagggttgaaagagaatgaataacggggcatctgccgccaaagaagcagtgaaatacttaattaagaaacaattacagaagcgcgcgcttctgttttttttatgctcttgggccggtttaattacgattgtagtatgtgtagttattgtctgtgcgatagggataatttctggcctatcaggttcagattcgggcggaggcggcggagaatctgcgataaacattgcgccagaagttgaacagtatagggcagttgtagaaaaagaatgtaaagcgaatgacataccagatttagttgatttaatactagcactgatcatgcaagagtctggtgggaagtcattagatgtaatgcaagcaagtgaatcaaaagggctgcctcccaactcaattaccgatcctcatgaatcaatcaaagtaggtgttgcaaactttgcttcagtatataaagcagccaaagcagctaaaaaaaatgtcaaagaaacggcgctgcaaggctataactttggaagtggatatatcaattgggcgataaagaaaagtggaggttggacaaaagaaaacgctgctgattttgctcgaattcacagtaacggacagcagcgcccaaacggaacttggatgtatggtgatcagctgtatgtagagcacgttatgaggtacctaaagccgaataacggtgaaaatggtggagaagttgaggtaataaagggtggaaacaaagttattgagaaagcaataaaagaaggctcggcttatataggaaggtccacttatgtaatgggtggggggagaaatcaaagtgacattttaaaggggatcttcgactgtagcagctttgtacattatgcgtttaacaaggcaggtttatcccttggaaacttagcctctacaacaacagatacgcttgttgtacgcggaaaaaaagtcaaatattcaaatattaaaagaggcgatttagtattctttgatacttacaaagtaaacggtcatgttggaatttatctcgggaatggagagtttttaaattgccaaaatagttatggtgttagcgtggcaaagatgagtaatagctattggaaaagtcattttaatggggtcgtcgtacgtattacagagtaaaggaggggaaccgaaaaagtgaaaataaaatttaaaactgtcggtgcaaaatataaagtttctacaggtgttattgccatgatcctgctgtttttcttgtccagcagggtcatttttgattcgccgtttgaagaagaaaatacaaaactaaacacccccgttagtataaataacatgactgtggaaatgacggatcgaacttatttttcagacaatcacatgcttgaaattgatttgatgatcacagattctctacaagatattcctccaaaattagatgcaattgttaaggaaaaatcaaataagagaaagaaatatcatcccgaaatcatcaagattcgtgatgatttttatgtgttgtttgtaagagatattccggaagattggacagcagtttcggttcagctgactgatgaaaatgatgaagattcaagctcaatcgggtcgagcaaaaagatatattcctcatctgcagatacgaaaacaaaggatgtttttgtgaaaagaaatcaggattattatgaagcaaaatatatcgatttaaagatcaaaaataataaaaaattgattcaagaagaagagaaaaaacagaaagaatatgcggttgaaattactcaaataaactctcgaatctcgtctttaaaagaagataaggaataccagatcggtaaagaaaaagaggaaacagaatcacaaatttcatccaatgaaagcaaaatttcttcaaaagaagaggcaataaaaacgagcaaagaaatgctaggtgaacttgaaaaacggaatgaattattgaagaaaagaaagagcaatctcgtcatcgaagactaaaaaaagaaacacttatttgaacagatcgttgcaaagtaatgtgcagaaatcgatgaaaaggagcgttaacaaatgccggatctcaacatcaaaggtctttcaaaagatacaatgaataggcttgcggataaagcgaggaaggcaggactttctcagcaagaatacctccgccaattgcttgataaacatgttgttgcggatgaagttgagggcgtgcgaagcgaattaggagaagtcattaaatctgtagcattcgccctcgaacaaaacaccaaagtacttaacgaattcatcagagtaaatgaaggatagcgaccgattgaggacgctgtccttatttctttttaaagcagcaaataagctggccgcagtgtttaaagcgcaaagtcttttctttattaaagaccgtctttaaaaagaaggaaaaatgagctgcaaagatcattttgtgctgtcatgtgtaaaaaagatattagaaagtgagggttagatatatggcaaaagtaaagaagcatcttacctttagtggtccgacagaatcaccgtatggtattgcttatattgaaaaagaaatgaaagcgaagaattgctcaaaaatgaatgaaacaattgaactgatctttgctgaacacgatgaaatgaaagcgagattatcagaacaagatgcacttgtcgagaaaatatttcagcgttttaagaagacgcttgacgttatccgtgtgcgcgccggacacaccgataaaaatgctcaaattaacttagagctttggaatgcatttctcatggccaacccgttacctgtgacagttttaacggaccagcatacctctgagtcagtatcgatggcaaaagaaaaagttagtaatgacattgctacatttaagcaaaggaaagatgaacagaaggctaagcaggaaatgcagaaaggtgaaaaataatggattctcctggcgttgtattagtctctaaatatgtgtcgggcaaatcaacaaaattttcgaagtatgtcaattatatcaatcgtgatgaagccgtccgaacggagaaatttcagacttacaatgtaaataaattagacggatacaatcaatatatggggaacccggaaaagagcagcgggatctttacccagcacaaagatagcttatcaccagtagaaaaaaatcagctgaaggagattttcagacaagcacaaaaaaatgattcagtcatgtggcaagatgtcataagtttcgataacaagtggttagaagaacgcgggatttataactcgcaaactggctgggtcaatgaaggggcaattcaaaactctattcgaaaaggaatggaagttttattaagagaagagcagcttgaacaaagtggcgtttggtccgcagccatacattacaacactgataatatccatgtccacattgcgctagttgaacccaatccgacaaaagagtacggcgtctttacgaacaaaaaaacaggtgaggtttaccaggctcggcgtgggaatcggaaattaaaaaccctggataaaatgaaaagtaaggttgcaaacaccctcatggatcgggacaaagaacttagcaaaatatcacagctgatccatgatcgtattgctcctaaaggacttaaatttcagcctagattggatacatacatgactaagatgtataaccatatctacgaaaatctgccggaagacatgaggctgtggaaatataataacaatgctttgaataatattcggccggagatagacagtgtgattacgatgtacattcaaaagtatcatcctgaagactataaagagctggatcagtcgttaaaagaagaaatggaattcagaaaatcagtatacggagatggaccaaaacaggtagagagatataaagagtataggaaaaataaacataaagaactctacactaaattagggaactccatgctgaaggaaatggccgaaatacgtaggcgtgagtcgcaatcaaaacaaatgaatcgctcaggtacctatgctcctagttcagtatcaaatagacaatgggatacaaagggtaggcgcataaaaagatcagatatcaataaaatcaagcacgctttagataaagattatcagagcatgaaaaacatgcgtaagtaccaacaaatgcagtatgaaatggaacagagccggtaggcaattctgaaattaaaggagaggaagccaatgatttttaaactagatcactatatcaatgaagagagagatccagattatttgctttttatcgaaaaggacattgaaccttcccgatttgaggaagagcttttaaagcttatagagataattgggtgtattcattttagatttgagcagcttgttagggatgatatttgtgtggcaggaaaagatatagtgttccttcttgagaagtattatggtttcaaaaacgtaacgtccgaatacatgttgttagaaaaagaaacaaggctgccgcgtgaggaatggtatgtttttaatgaattcagagttggcactaaccaagtgcccgtgtttcaaatagatgtatataaagcgcgggaagcatgctgcggaccggaatacagaaatctcatgataaacaggctgccacttgataaggaattcgataatgatattgaaaagctaggagctttttatgttggtgaacagcattaaaaattaaagaaaacacatgtgagatcaggataaatcctggtcttttttttatgactataaaagggggagtttaaatgcctagagtaagtgaagatgtcataaaacaagcagctgcagttgatattgtaggcttctgtgaggccaatggttatgagcttgttaaattgagcgatagatggtatcagggcgctgaacacgatagcttaatgattgataaagagaaaaacagctttcagtggttttcccaggggaagaacggcaattcaattgattttgttcgcacattttacggaaaaagcttccgtgatgctgtatcaatgctcactgaaaaagactataagcatacaaaagaagttaaagagcagccgcaaaaagaattcgtttatgacatcgttcatgataactccacagaacaagtcgaacgttacttgactgaagaaagaggcatcgataaaggaatagtaaatgcactaatagcgaaaggattactgagacaggataaaagaaaaaactgtgtgtttgtttgggggaatacaggcaagcgtgtaggtgccgatcttcagggtaccattacaatgaataaagacggaaagagaacgacatttaaacaaattaaacccaattctcagcggaattatggctttaatgtctcattaggcgtccctaaaaaactttatttttttgaggcacctattgatctgttaagttattggacaatgtataaagaccaattatctaattgccgtctcatttcaatgaatggagtgaagaaaaacacggttttcaacctgataaagcatacaatgaaatcccgtggtgtggctccgacagaaggagtatacttcggagttgataatgaccatgctggccacaaatttatggatgaaatacgacaatatgagttttctgttaaaggggaggaagtcaaatttcataacttaatcccggcagacaatcatattcccaaagaatatttagaactgtatcaaacatacggcagccaatatggggtcgattggaagtacctagctgctattcataaagctgaaacgaaccttggaaatacaaatgagattacgaacggttatggttttggcaagtattttggtgctaaacagctgcctagtgaaaaaccttatgagatccaggtgccaatagcaatagaagaagctgccagggcgttaaaagctaacactatagatggaaaaactgatataggatcagttttaaaacaggatgtaaaagaggttgatctgactaatcaggtgaaaatgcaacagaaagtacaactttattacgacaactataatgatctaggatatctgccggtggaagaggtttctaaggattggaatgatgtgctgaaggtccgtagagctgcttcaaaacatcgcgaaaaaacacattctcaaaagcaacataggagcaaaaaaaatatgcttgttagggggtgataaaacaccgatttacctgaattaatcaagggaaaaaaaggctaaaaggtatcttcagtatcgctaaaatggtataatatattatagagaaagggaggtcaattgtatggaaaaaataaaaacaattgagcaagctcgtgagaaaatgaaagaactgctggctgacccccaatataatcgtccggagaactacccggaacgaaacgctgacgggactatcctgttagatgaaaataatgaacttcaccaggaattaagataattggctgaaacagatccaaaaaaattagagctaggcaatatacatttagcgataactgaatttagagatgggacaggtcgtaaagcgcggcctgtccttgttttaggttcaaagaaatccattgaaggtgctttcgagcctgaagtcctgatcgggtacatcacatctaataataacaataagaatttctccaagtttaagtatccgattgctgactggaaagcagctggtttggataaggaatcatgggttgttttgcaggaacgggaactcaaatggatgaatcacgagaaggattttcttaaacacatcggattgctgacggaacgtgatacaataggcgtcctgaataaatttatggaagtccgagaattagaacagtcattaaagcaagaggctgaaaaatctaagccgcaacctcgaaagggtaagatgcaagtgactattcaagagaatcctacattgaagcgcagtagtccaagcgcacaacgaagaaacagcagagaacggtaattttttttgaagacaagctccctcacttcagggagcttttttatttttcttattgtattaaatgctgccggttgcggaaacccaggaagccaggtgcgttgcgccgatgatgcggaagctgaagaagtgccagtgatccaggagcgagaggataaataacttatagagctgaatattctcggacacattctttcagctaaagaagggagataaaaagttggtaaataaagaagtaagtataagtgatgaacaattaaagcgtatagggctagacttattaaattttggtctcgtatatatccgttcaatatcaggtgctggacattttcctaaaagggaacaagcaatagtaaatgatgtgtgttataggatgtcggatgctttgcataatctccctgagcacttaatttattttaatcgcttgttaatacttgacgaattagagaaactggcactaaccgtttctcgtattcctaaaacaaatatagttcaaaatccgactctacagttaatagttgaaaaaataaagctgttgtctggagattcttgttgcaacactcaataacaagtgcccttattttgttactttttttatcattttgttgtttgcattgcaaactgaatatactgagtatatactggttatataatttatacgttagtcatctatatgatgaccaatgtaaaaaaaacagatgtttttgcataaaaaaataccggagtgcgccaacactccggtctgtacacaagctgtccttaaggggctggctcgagtatttttcctaatagacttatccctttaacttttccagagctcaagggaggtctattttttgttttttaaagtcaacacggcaacaattaaagagcccaaaccaattaatgatgattggaagctaataaataccattagagcttgataagcttcagttgacattttatcaccccctttcaggggccagcagatcgctattgagatacacggcaaatgtacaggaataatatacactagacaaccatattgtggttgtctttttttgtatcttaagtatagcaagctatggcaaaaacacaatatatagattagtgttttcacaaattaaagaagcatttctcactttcatataaagacaataagagcttctcatctatttattttagcatggtcattgtcccaccgtataaagttctttataatttgatcttctttcaagactgccgatatctttagataaaggagagatataaatgcttacagaaagacaagcgttgcaagatcgtctggaaaaaatagacaaagatgaaatcactttgatcaaggagtatcagaaacaacgaaatcagatttttgagcgtcttagagaaatcgatagagaagaatataaaaaccttcctgatcttaaacaattagcctcgctagaaattcatcaaaagtcaaaacctgaaagagacataagaaaacatgttgccgttaatattttgaaagtcaatccagacggtttgtctgctgatgaacttaggagtaagattgagaaagagacaaatatgcaaatacttaacatgacaaattttatgagatcaattatggagaaaaatccttcagtaaaaaaaccacgaagaggttattatagattcgaagaaatgtaacacaatgttattgtgttacattttcaaaagagtgctaatcccttatgtaccaaggggttagcactcttttttttttgaaaaagttaaaataaagtataaaaatgtaacacaacatatgttataatgatattgtgttacattttcaaaaagaggaaaaggggtgaaaaaatggatgttcagtattgggaagtgaatgttagtcgtaaagaagctgctaccaggattgcggagaaacttaacaaggttaagtttttgtttgacgctgggatttctgatactccaagaggaaagtgtctctacataaaatttgatgattggcacctggaatataccgaaaaaacaagaaatggaatgatgctttttctcaatcagttaaatagcatgataagagataaatcattggttgctgggtttataaatgatctgaacattatagatttggaggggaagattaaatgttgaatagagtagttctagtaggaagattaacaaaggaccctgatcttcggtataccccacatggaacaccggtcgtcacttttactttggctgtgaatcgtacatttacaaaccaatccggtcaacgtgatgcagattttataaattgtgtggcatggagaaggacagctgagaatgttgctaattttttaaagaaaggcagtatggcaggagttgatggccgtcttcagactcgcacttatgataataaccaggggcaacgtgtttgggtaactgaggtgttagctgattccgttcagtttttagaatccaagaacaagaatcagaatgagaccaaccctggatacgatcaaggatttaaaggtcaaagtaacagccgggaaggttttgctgatgttggtgtggggagagatccattcacaggtggaaagcctattgatgttagtgatgatgaccttcctttttaatgacacgaaaggagaatttagaccatgagagaatatttatcgtttaccggtatttgcattgcttttctaatgtttttgtatgtgggtttctattggatggtacatgagactgacgagacccttacaaagatggataaagatatcaatagtcttatagaaaaggcagctgaagaagcaagaattgagaaagaaaaagtgttaaagaaggggaagaagctggatgctttagtgattgacaaatattctactacagattcgagtatggattttaccgtaacaccggttgttataggtggtggaatttatatgatgtctggagctacaccaggagtaacaactgagaattattacattaaaatttatgcagacgaaaaaaattatgacataactgttcctaaagaagtttacgatcaaaaacaagttgggctaagaataccgattaaactttataaggataaaatcgaactactataaccctccgggatcagtcgccaaacaggaatcccgaagagttaaggaaatggggctgcttcagcccttaattaagtataaattattaagcaatcgttgaaaataggaggcgctgttatggaaagaaaagagaaaaattttttaggatttaccgtaagtattgttgttggtgctattgtggcctctttatgcataattcaagcgattttcccaaatgaatttaaggcattcttcattcaacattctattttctttaatattatgggtggattccttgtatttattgttgccgtgatactagggtttgtaacctttataaacggaagatactaacaggcggggatattgaaaaaactgttcaactaacagcagcactattacaatagaagtaatgcaaaaaggactgtgaatttagatttcacatgacttaatttaaaacgaagaggtaatttgtatgaatttagttgaaccgatccgaaacagaaaagatatagacaacatgaaaaagctactttattcgatgaatgaacgtgacgccgtatatttcattatcgggataaacactgcttttcggattagtgacttaattcatttgaaattcaaagatgttattgacgaaaaaatgaagcccctagattactttgaattgagagaaaccaaaacagggaaacacaacaaaattgccatgactaaaggtgttcgaaaagcaatcgttcaatatgttcagcaccggtatgaagggaaccttgaccattaccttttcaccggccagaaatctaaagataagccgattaccagggtgactgcctggcggaatattaaggctgcagctgacacaataggcttaaaaaacattgggacgcattcattgcggaaaacctttggttatcatcaatacaagaatggaactgatattacgctgctgatggatatgtttaatcatagtagcgcgggcattacattaagatatatcggaattacacaggaccaaaaggatcaggctgtgaagtcattagacttatgatttgactactaactaacagggggaattcatgatgtcaaaaaaaataaaatacatgttcgccattgcgctggtgattacgctaatggttttattcaggcatattttattccttctgttggtgaaaatggtcttcggcgctttactgattttcgttggtattgttggtgtgtatgctctatttagattatttgcgggattaataagtgtggcacttgtggtcgcaggaatgtttcttatttttaagatcgttcaattggcttgtgcatagaaaggagatagcatggaatatttattattactaacatcattgttacttttgcctttagctgcatggggtccagaaatttttgatggtttaatgaatatctccaataaaatttctgatatgagagagcttcctaagaagtacaatacgagtaaaaagttaattagagattatttgaagatacaaaaaaatttaagtcttaaaatggatgctatcgtatatcgcccaaacaaggatgtaagttttacgacactggtggataatcttaaagatctgttggatgttcttagattagaggctccacgctttgatcattctaataagaatgatttattggtaaggaattttcctcaagcttattataaagtatacattcagcttatacgctatgatgactctttgaaaataatatttgatcaattgatatctctaatctatggtgattatgatgacccccatataaaggagattaaagctcttagagatgaagtgacggatattatcgtgtcaattagaagagaagccgaaaacacaattaaaccttatcgtagagagaaaaacgaattatttaaagtcaatgttaaacatgctaaagaaagaattgaatttgaaaaacagttcataaaagagcaacgcgcgttaaataatgccggctcaattgagttgaataaaatataagatcgttcttaatgacgcgtattgcagtggatagtcaatctaatgaaggggtttaagataatatgaatgagacattgtttaatatatttgcaggattgtcttttattttcttgttgttaagcctatttaaaaaatttgaacgtgtgtttatctctataggagcaatatttctaataatggcatttagtaccggagggtttggcgaagcacttcgttcatggttaccagttgatcaagatgtacaaaatcaaacactctcggttataaaaacattccgtattcatttttatataatattgttttttggaatcttgggagtcattatcagtctatttgttcggcataaaaggaataattctagtgtaagtgaagaggagtgaatttgaaattgaatttaaaaaaagttatcggggtaatcctgatgactttttttgttgattaatttcctatagagcaatcaagaggtataattttcaatatggaagtgagagggggagagcacgctggttattgataagacgagaatatttatcagttcagcatacgaagagtccttaaagacaccgagaaaaatcatcaaaaaacacttagaagaatgtggccatgaggtacccatctttgaagaagaagattttggaacatggaagccggatacaatgaagcattgcatcgaagtagttgagaaaagcgacattgtcatattactgataaacactaaatcaggtgaagaaccggaattaagatgggggaatgtaacacctacatacttggaattccaagaagcttggaaaaagaagaagcacattttggttttcgtaaatccggatatcaaaaagaggttctttgaattaaaaaaggattttgactcactatataaccaatatattgaagagaaccataggccgcctgattcaccctttgatcctttcgaaaactggatcgccagtcaggatggaatggttaaaagacatttagaagctgctgatccttttgtttgggcatttttatatgacatatatataaaaaggtattggttgtatgaatttgattatgcacaatcggaaaaagaggctaaacaaattgctcaaatgatcagcaattctttaaagacggttgttgactttatccctaggttagacgagttaactgagattgaagagcagcagtcatatttagtagaatacgccgaacacacccttactatgctccatcaaagaaatttaatattgaataaagagcaacaagattggtcaaactttttaaaacaagggattgaatttcttaaccacagttacgaaatcatacaggctaaagatacaaacccagtagtcgttaatcatatcaattcatgttatgctgcttcgttatattctcaggatggagaaacattaagattggtcggaaaagcaggagatataacagctccggaagtatttgcattatacgaagagggaattcatgttgttgatgccttcaatcaaggtgaacgattaattacttacagggaagataaaaagacattctacatcactgaggccattgataactttgttctatgccttcatttttcacttgaagaggattggaatgtaaagcgtgctgaagcatacgcacaagaggttgaatgtgctataatggataaacaccaactctattttgaatttttgaacttgctgataggagggagcactaatgagtagagaacttgcgaattacagtagctctggctcggttgttgttaaacgttccccagctgtaagggcaagaaaagttaaaggttctgccggaactagggctagaaaaattacagccgatggtaagtatattccttctcaaaatctaagaagaacaatttctaaaatgaattcgaatgttcggtctttaaatgatttattgaataagtcaaatcaaattaaatcagatcaggaaaatcgttaaaatagtaatcgtcctttttattaaaggacgattttttgtttataggcaggaaaagaccgtgcgtcagtatcctctatacagctgaaggtaagatccggccgcatccggaatccaggaaagcaggcgcgctgcgccggtgctgtggcagctgaagaaagaggtcgatgccaggtatcggagcacctggaaatacggtgaggcccgcgacatccccaatcttatacgttagcgacattgaaaatttccgaagagggaggttgaaacgttgataaagaaaggttttcgtgattgtaacagtgtaacaggtttactcgttaacaaatttactgtgtaacagtgttagtgggctattttattttttttgctgtggattttttaaaaaaagagtgggggagtagttatgtaatggagaggttactctctccaagaaacgaatgaaggtaaacgaagtttcccgtgtttggtcataaaacgatgtttaactttgcacgagacaggttcaacaaaaacaaaatcttcagtttcagactttaattttttcattgaatgaaacttatgtcgctctgactttggcataaattccatcatgccagcgggcgtgccatcttggtaagacagcagaaattttatatctttacgtgtgtagccgattatcagcacttcagtaaagtcataattaatgactttaatccagttcttagaccgttttccgatttcatatactgagtttgctttttttaggacgatgccctctaatcctttttctttaaccatattgaaataggagacaccatttccttttatcccttcaagtacaaaagcattcggatggtttatttcaagacctttaagcacttctttacgttgcgttagtgggtttgatgcgatggattggccgtttgaataaatgacatcgaaaatgcaatatacgatcttatgtggggacttattggacataaaccgttccataacagcctcaaagtcaggagatccatcggcaccggttacgattatttcgccatctaacaccgtaccgtcaggaacatctaaattcaataactcaggaaacttgctgctaacttcattgttgtgacgtgtataaagctttatatgattattgaattttgatagtacaatccgtataccatcaaatttaagctcactgatataagaatcatcatcgaatggttcttttgtggattcaagcagcataggggatataaacaaaaaatcacctcccttatgaaataataaaggaaggacgatggcctataaagtcatttgaacctggtatataatgcaaactgtttgaaacaagaatcaccggaagctcgaagaaaattggaaacagacaatttttcttttcagaattttttacatatgctatagttgctctaaagttaaacattaaagcaaaataaatggttcctatatactttggcagtatctgaggctaattatatgataaggaacaagcccaaattaggggggagtgaccaatagtcactctccccttttagttactaaatatattttgtttctttaagacatttaaaacaagaattgatgttttgttataacatcaaactgataaaaataatgaagagacatcaagtaaaagcataggcggaacgtcagtttgttaggatttcattaaaaagcatcatcggaattgtaacaaaaaaaagtggggataatgttggttactacggaaatttgaaaggaggtgattgtaatggttgaagggctgattgttctagcgtttttttcgctttggttgatcttgttaaaaaaatagacctcccgcaagccgaaaaatctagagggaagtctaccaaaatttaagtttccactgtccagggtattggtagtaccctgacagggaaatccctgacattattatttccaatatgtaagaatttatgctcgatcaaataaggaggtgattgtaatggttgaagggctgattgttctagcgtttttttcgctttggttgatcttgttaaaaaaatagacctcccgcaagccgaaaaatctaaagggaagtctacaaaaatttaagttttccactgtccaaggtgttggtagcactttgggctacttatcatgttatcaaatagaggtattaatgtcatctaacaaaaataaccccggatggtcatgtccggggccggtagaaatcaatcctcaagcacaaagattgattatatgtaatgatacacatcgtggtgagatatgtaaaccaggatgttacttggagtatatcttcattttttcattggtctttttgccgttcttaatcttatccaggtactttttaagaaaagaatcatatagactatccggaatatatccaagtctttgcagcaagagattttcaacgatattcattttctttgtgaggaattgataatcattcctggattcctgtgaatcagtgttaccggtcgccgccttcttataaagttcattatacttttggctgcgtttttgtctgataagctttaacaagcaaagcaactcatatgtgtgaaaagtcattaattcaggtgtagtcttgtaaaggtcctcttcatcggcagtttcacggaagggaactgttttgcggctgccatcttcttcggcgtcttttatcttgatcatgcagaattcacattcataatagttagattcgttttcttttgctacggggctaccgcagtatgggcaagttttcatttcattgatctcccgtcagttagatttttaatgttctcattaagtgaattcattaatgagtgatgtttttcgaggaattctttcatttctttagtctttttatctttaaatgactcattggcggataaagcaaatgaatagtatcctttaagcaattcatttactttatcaatttcagcttttaagtccacaacatcaggaatcttgcaaaagttttctaaggtggctagtgcataacaaatagattccgaaaactctaagattatatctttgttctgtttttttaataactcaataggggcccacactttagccttgatttctctatttaacagagagcatttttcagaacttatactttccttttttactctaggtctgaagtagttgtattcaacgtatttcagcaatcctaaaaattttttgtatctagttatttcaatactatcacgaggatgtcccaaaactttaaagtaagatggcgcctttttgctatcggtaaatgaaaaagatctacgatacagttccagttcatcttctggatcttctttatctgtggtataggcaaaacatacaagtctaaagtcaatttcttgataaatatctgtgccatacgctcttacataatattcattcacctttgcgttgcggaattctgccccttttctaaaaaactcgtaaacaacaccttttttaaagccatacaaacgctcataaatatcgttaagacaaaccactgtatacagatattcaataggaagttctttttctaaaggaagtatagttttacacattgttttattcacctttcttattattccataatcccaatttctttttctttgcttctttttcagcttgtttgtattcatcttcatatttaatatttggtggaaaaacagctaaacgagcatagcccttctctaagagaattttgttaaatgaggtcccgtcctttaaaaatacgtatgccaatagtctatcgtatttatcacgcttttctttgtcgtattccagataaacactttgattctctaacgtcttttttgaaaaggctgaagcttcttttccataaggctgcactgcttttgttggatggactgtttccggagtatcgaccaatattaaacggattctttcctcagtaccattaacatcggcaataaatgtgtctccatctataacgcgtctaacagttacctcaattttatcagatagatcaacggtcttttcagttgttccagaatggctgctgctaacgccctggcatccactaagtaggatgaccaggacggccaaagcttgcattaactttcgagttagcatgttctttctcctttgagcgtttttttggctgagaggaatatggctgtaattttaattacagctaaaattcctgatgtgcctgccggcaggtattgaataaccaggttgtgctgcggaaatgtacccgattctgtgaagacaatttgattgtcagttttattgaatgccatagtattatagtctaaatcttcagcaataaaatccgtttctggtagagtgatagtacggttcaagtgaggcgttagatgatcggacacatccaaatgccatgacatagctttcttcatgattcattctcctttttttaagacttttttggttttgcttggggagccaatcagcattcacagtcgaaaggacacaaggggttacgagccgttgaggggtgttctgtagccctttacggatcgttaagaccaatttatttgtggcagctgcgggcagctgtccgtttacaaaaaaattggcggcccttgtgtgcttttatgaaacacggatagtaacgcggcgggcgtgcccggcgtgttgcttgccgatgttgaatgtgaaatgctaaagcccccggacagcttcagctggccaagtatgggggcgtttggctgagcaaaaacaaaaaaggcgtctaaaaaaaggatttaatcatgccggcggctgccggcattctttttgcggaaatgcgaccggggctttctgggagcctttctgcttcttttgggtttaagaggctgctttagcagcctccaagcaggctcgatgcctgcgttttaatcaaggaaaactttagttttccgaccttgcgtaaccggcaaaagccggttgcgattttagccgcaacaaattttgcgcctaatttgaactcacgagttttaagtctttttcgtgaactattggaccatcttccacgtcccagaaagataaactttcatcctcacgtaaaagagcttccgtatctttatagtaaaaatcaactgctacgtgtgacatctcctcatcttctttgtcatgccaaataactttccctattgtaccttttgggaagtgcccccatggtgaatcgtgatcaactaaaagctgtacttttgcaccttttcgaaatgttttcatgttttttcctcctttgatttttgctgtccataagtaaatgcggggggaccagccccgcgagtttttccttgtgcttgtgtttttgattcctacctgtatttaacttgccgtacttatttgatcttcttctgtattttctaaaatatagtcaacagctttttgggcttgtgcagatgcatggaatatcaggcggttatcgtcttttaatgcagaaagccaggatttgatatagcttgcactattctcaatggtattgttttctatcccggcaatgccgcacagcatagctgcacccatttctgccactagctcttctttagaatatttctcgtcaccaaatgtaccaaaggttcttgctaggcgacttttatggcctgtactgtgtatcatttcatggaaaagagtcgagtagtattcttctggcactttaaaatcttgtattggcggacaattgattttatcgagtgttggaaagtatgcagcttctccaggttcaaaggtgtaggttggaccattgggatagttattgataatttcttcagctttttcaatgggatcgtgattatacgtttcttgttttcgtttactttttagcccggtacattgtttattgatatcccatacgcggtagtagataggctttgcaaatttctttttttcttctgtttcttcgtcttcaaactctttccataaccagaacacaatgatatgtgagtttttaaattcttcttttttgatgcggccgccagcttctaagatttgttttttagaagcgtattccccaggagggactaaaaagttattgataccccgataaggcttttgtgttttccagttaactgctgcacaggaatttgtccagggctgatgccaaggaacaacacccttttcaagttgtgcaataattttctccgtgatgatttcataaactgatttccccacaatgtgactctcctttttttaagacttttttgtttttgcggaggccgaattgcattcacagccaaaaagcacacaaggggttacgagccgttaaggggtgttctgcatccctttacggatcgttaagaccaatttatttgtgacagctgcgggcagctgtccgtttacaaaaaaattggcggcccttgtgtgcttttatgaaacacggatagtaacgcggcgggcgtgcccggcgtgttgcttgccgatgttgaatgtgaaatgctaaagcccccggacagctttagctggccaaggtgggggcgtttggctggacaaaaacaaaaaaggcgtctaaaaaaagggtttaatcatgccggcggctgccggcatacgttttgcggaaatgcgaccggtgctttacgggagcctttctgcttcttttgatcttccgtcctcgttcactcgtgaagaaatggccaggaacaatgcagctgttgcttcaggatccgccgcaggcaatccggaagcttacagatgtatgttatcgggcattttagagggaagcgagatgccgcggaatgttggccggcgtttttggccggcttacagtccgggagcagacccgcagggggacccaagggaaatttttaaccatttttagaagtagatacgcaacttatagtaactgatgatgtccattttgaaagaataatacgcagttagaattagaagaggttttcaccataaatttgtgccattttaaaaatcgcttcgcagttaataatgagggtagaaattttcccttaaatgtgcggtataaaaaaagtgcgagtattatctagtgaacatgtaagagaggggtttgaaatttaatgtcccaaaataatagcttaatgcaagttatgaagtgtaaaagaaaaataagactaatcgaaggaaggaggttaaacggaatggaaaaaatcagtaagggagaaaggagaaataatatgaataaagaggaactgctgtggatgttaaggcttgtcttaattacaaattcatttacggccacaatattgtttggtatgtttaaagttattttgattgctacaggtaattaaaaagatcagcttaaaaactgatctaaaagggtgactgaagatgttccagcatcagcagtcatcatgatataaagttgttgtaattatagcagagaagatataaagaagaagcttacaaggttttgattggtggtttgcgcagcaaaaccaccagagaaggttttaatgtttttagaggttgctttagcaacctccaagcaggctcgatgcctgcgttttaatcaaggaaaactttagttttccgaccttgcgtaacgagcttaccgcgctatgtagcgcggtaacttctttttgttatttgagcagttcttgttgcgtaattaaccaattttcaattttttcaactacttcacaaaaatcttgatcgaatggaaaaccctcattaagtttgttaaacgtaacatcatcagattcatcccataaatcagaaatctcccgtgcggaagttttgaatagtgttaaggcgtttaataatttgttttttgtcattgcaaaaactccttgctgaaccgttcaataaagtatgacggtagtattataattttttcacttcaacgtataatgaaccttccgtgattaacgatttaaagctttcgatagcttcttcggctgcttcttcttctgaattggcatctacttcaatttcgcaaactactaggtactccatattgttcccctccgaatttatatagagggacaggtagacgaatcctgtccgatttgtgcttgtgtttttaatctctaccgagtttctattcaaatatagcctttgcggccctatatgcattcattgttaattttctttgccaggcttgtgagtgtggtgaccatctaaatgtgtttttctttaatttatcttttaattgatcgtcgggccgttgatcatcaggaaagataatttttaatctgtcgctttcttcatcagcgactacgcgacactgttcataagtcaaagtgggatagtgcggctttttttcttcagcttgaaagagtttatagatgctgtgacgttttgtgaaaacttttgtcatgccttctgcttcaaatatcttgtataactcttccttgttgtgtccttctttgaatagtctttttaatttggtgacgagactgtttttgaataacgtaatatcatatccaggcattttaccttcttttattaggcggattcttatacaatcttttctgaattcagaatatgcctttactgctttttcttcgggcttctctaaggagccaagatgtttctttgtgttttgaataaaccgtgtcatcttttcagttgtttctcgatcataattgtcttttcgagttaattccttttgctttctttcaaatggatagtttgcccgtccggtaatcaagggacttggtgttttgatcatggtaagtgatttctccattcgctgagttaaaaatttttcaaactccatcaacctatttagaaaataatctctttgatcttcattttgaactagaggtgctagatcgtttttaaatttgtttgcataatactgaatttggtgatcgggattgtatttgtacatgtgcaactcgttatatctctttgtgatttcaggttttacgtacgtttttactgccattacatagacactccttttttgttttcatattcaatcatttttaatgctcgccaaaacttaacatcaggaattcgtaaatcttgccgtatgtcagacaacagttgcaatttgtctagaactactttgcatttttcttggtagagttgaacttcaaatggacagttagcaagttctttttcttcctctgttaatttaaggtctagttctaaatctgtaatgtatctggctaataccagcgctatttcttgtttagtcactcattttcgccccttgattaaaaattgagtggaaggggagaccaacccccaaccgataacccttgtacgtgtgttcttgatttctaccgtttttattctgtaacttcaaaaaaacgtttaagtggaggcaaagcccacccatcctttttggtttgggcaatagcttttttatacattgcttcctcaaaagcatcacctaatcgtttttgctctttttggtaatcaccttctaaataaacatttaattgataatcaccaaaatcgatcttgactatgatcattttgtcctccttttttaagacttttttgtttttgcggaggccgaattgcattcacagctaaaaagcacacaagggttatgagccgttaagggatgttctgcagccctttacggatcgttaagaccaatttatttgtgacagatgcgtgcagctgtccgttcacaaaaaaattggcggcccttgtgtgcttttatgaaacacggatagtaacgcggcgggcgtgcccggcgtgttgcttgccgatgttgaatgtgaaatgctaaagcccccggacagctttagctggccaaggtgggggcgtttggctggacaaaaacaaaaaaggcgtctaaaaaaagggtttaatcatgccggcggctgccggcatacgttttgcggaaatgcgaccggtgctttacgggagcctttctgcttcttttgatcttccgtcctcgttcactcgtgaagaaatggccaggaacaatgcagctgttgcttcaggatccgccgcaggcaatccggaagcttacagattgcggaaatgcgaccggtgctttacgggagcctttctgcttcttttgatcttccgtcctcgttcactcgtgaagaaatggccaggaacaatgcagctgttgcttcaggatccgccgcaggcaatccggaagcttacagatgtatgttatcgggcattttagagggaagcgagatgccgcggaatgttggccggcgtttttggccggcttacagtccgggagcagacccgcagggggaccccaattaatcttgataacaacggatcacaaatggaaaaaaggatgtgctatgctttgaaatataaagagggggtggtgtcaaatggatacaaatgaggtactacagttgttaattgctacgaatggaactacagcaacagttttagttgggatgttcacattaattttaacggcacttaaaaagtaagatcagtgtattaaaacacactgatcagcagaatgattttgtaactgagatgtggctgcatcttcagttacgctcattatagcaaattgattttggttttccccctgtttttgcgctagcaaaatcaggggggaggttttaaaggttgctttagcaaccttcaagcaggctcgatgcctgcttttaatcaaggaaaactttagttttcctaccatgcgaaccagcatgattttcatgctggtttgtttgccgtaatatctattaacattaacagcaaaattcagatgtaacattatcggtgtaaagcacttcattttctccggcttcttctggaaaatacgtttccccatcaaactcgtatcttttctctgaaaggacgactgtcataatagatgaaaagcagtccgggtcagcgtggattttatgcatttcctcgttagttagtttaaatgatattcctgcccgtccccaaattgttataaagccaggttcttgggaggactttttagatgattccatgttatctcactcctttggaatggggtgggtttcctgcaccgcagattaatacgttagatgtcgcaattgcatcctgtagccagccggcagtgtcatccatgatgtactcactttgaaattcagacagtgagtcatagccgtgctgtttcgctttactttctgcccaatcgctgggaactgtaaaccaggcacaacctaagtgatcatttatgccgttctcatttggtattaattcaccaacgtaagtgtagattgtggtgactttcgccttttcatagtttgaaagctccgcataaggcgggagcgatttgtcttttttggcttgtttccacatatataatagatcgattgccgatatctctgaaagctttatatagttcgcttgtgtgttttcgtctacataacctaagtcgtgaagatcaaagcaagaatcaagagcttcacaaagttcttcaaaggttttgtagcgagtgagaatttcatagatagttaaagatttcattgctgttatcgtctcctttggagattgagggcagggggaccaatccctgccaaccaatctgtatgcttgtgtttttaatttctaccgtttttcacatttactcgttcataatcgaaatcgttgctgtttggaactaatttttcgcctaaatgctcgcattctataaccttccactttagcggagaaaccagtctttgtaggtatcccatagcgtttgcttcggtgtcaggaacaggcataggaatgactattgccggatcgccttgttgtttttcaagagttgcttgatatatgtcaaaatgcacttggtttatcattttgataacacccctgtatttgagatttcaaactgttttctatggcagtaagacacgtttggaaagtaaactcattctctatatctttataggtgaaaacatagcctatacggaaaaaatgatacttaccgttgcgtttaaaaatagattctacgaaacaatcaaattcatttatcccttgttcgtcagaatcgcaatacatagcaggctcatatgatatgaactcattctctgaaaagaattgattatgatccatgaaattcaaaattactgtatctatgaagtcgcagaaagtgccgcaaatagcttccaaactttcttctgaatgactttgtaacaaggctttatcgaaaggtatagcttcaggtatgcctgttaatgcttggtactcttctttggctatttcaagaaactcattgagtgacatagaaccaactagattcacgtctgctgtattgacattcatttgaccctctccttttgagtttttaggaaaatttactgcaacaaactacaccaagaaacgctatggcaattagtaaaaccaagatggaataccttttgccttcaccttttgttctgatagtgataactgataaaaagccaaataatgaaagtgctattatcactaaaatgatctcttgcatgtgaattctcctttttttaagacttttttgtttttgcggaggccgaattgcattcacagccaaaaagcacacaaggggttacgatccgttaaggggtgttctgtggccctttacggatcgttaagaccaatttatttgtgacagctgcgggcagctgtccgtttacaaaaaaattggcggcccttgtgtgcttttatgaaacacggatagtaacgcggcgggcgtgcccggcgtgttgcttgccgatgttgaatgtgaaatgctaaagcccccgggcagctttagctggccaagaatgggggcgtttggctggacaaaaacaaaaaaggcgtctaaaaaaagatttaatcatgccggcagctgccggcattctttttgcggaaatgcgaccggggctttacgggagcctttctgctttttttgatcttccgtcctcgttcactcgtgaagaaatgaccaggaacaatgcagctgttgcttcaggatccgccgcaggcaatccggaagcttacagatgcatgttatcgggcattttagagggaagcgagatgccgcggaatgttggccggcgtttttggccggcttacagtccgggagcagacccgtagggggaccccaaagtaaggattcctgaaaaatcctaaagaaatctaatgtaatcgatatgagatatagctctttcagctggactctgaagggttaggggtgttgaaaggggtttgtaaggctttgtgttaacaaagccttacaagaggtttttgtggttttagaggctgctttagcagcctccaagcaggctcgatgcctgcttttgatcaaggaaaactttagttttccgtccattcgtccgccaaaggcggcgaaaaaaccaggctatttgaagcctgattttacaatgttattttgaccatatttgtctgtttcggctgtaaggggctgtatcgtcaaaatgaagtgtttcttttagtctaaaccctaatttttcaacgtatctaaggcgtttcttcatcccaaaaggataatcgactttgatttcactagctgcttccaggtgtgctgggaggtctttgtaacgactgcttatgattcttccggaatctgctgtaattggtttatagatagttactgaattatcgagtcttacaagtatcatcatgtatcgctcctttggaatggggatgcttaagctatgaggttcccgaagattactgttccgaaaaacaacagtccgattaaagaaagtgatattcgtggactgactgctataattttgtcatcgaatacgatgatctctccctgggattcaagttcagcaatatgagtcatgaccttatttgaatcgccatattttaatagtttgctgattgtggtatactttgattcacgtattgatttgagcagtgattctttggtcggggtcacatgctctttttttattttccgttgaattgcttgtgctgcattcatattcattctccttcatcctccttcaaaatagttagcccactttcacttttattttccgttgctatttcaaaaatgagtttagtttggtcgtacgtatattcactcgtgaaggtactgatatcagggatatcagtgaatctgcggtttagaacttcttctaaccagtcctcgtaaacacaaaatcttacctgtgtttcagggtattcattggcggacgctttataagtccaaaaactgcagtacgcctttgactgggttttatctagctgtgattcgattgatccaattaggtcatctaatattgtccatccttcttcaacgcttctttcttttaatgtttgttcaaagccattggtaatgcaggcttcaatattcttctcagtgccaaggaatcctttggattctaatgcggatttcaggtcttctttatgccatacaatagatgtgaaaaacatatgtaacagctcctttttttttaagacttttttgtttttgcggaggccgaattgcattcacagccaaaaagcacacaaggggttacgatccgttaaggggtgttctgcagccctttacggatcgttaagaccaatttatttgtgacagatgcgtgcagctgtccgttcacaaaaaaattggcggcccttgtgtgcttttatgaaacacggatagtaacgcggcgggcgtgcccggcgtgttgcttgccgatgttgaatgtgaaatgctaaagcccccggacagctttagctggccaaggtgggggcgtttggctggacaaaaacaaaaaaggcgtctaaaaaaaagatttaatcatgccggcgcctgccggcaatcgttttgcggaaatgcgaccggagttacgggagcctttctgcttcttttgaacctctgtcctcgttcactcgttaagaaatggccaggaacaatgcagctgttgcttcgggatccgccgcaggcaatccggaagcttacagatgcatgttatcgggcattttagagggaagcgagatgccgcggaatgttggccggcgttttgggccggcttacagtccgggagcagacccggaggggaccccaaagtaaggatttctaaaaactcctgaaagaaatgattaaatgtaatcgatatgaggtgtaatgtgaaaatcaatctttctgctgagctgtgaaggtgttaggggcgttgaaagtgtttgtaaggctttgtgttaacaaagccttacaagaagatttttgtggttttaaaggctgctttagcagcctccaagcaggctcgatgcctgcttttaatcaaggaaaacattagttttccgtccatccgagaacttcaatggattgctcatagtcgatgacgccggctgtcctcgaagcaatcagggtacttattctgttttctttctaaaaaggatttaacttttattgctatatagtcaaatagtagatcaagtgctttgttgattaaccattcaattaataagacactaagaatatatttcatataaaatgttcctccttacccgtgatatatataaatatcaatttttcaatacaaagacttttatggaattcaaagaaatatttcaaagaaatttgatagcagaattatcaaaatttgggtaagattgaattgttgagtttcatttaagtgtgtgaagaaaaatgctgaagatatgctaaaaattaccgatagaaagtataggattggaaagagaggtaggcatgaagaatataaagcatattaaaaagatgaggaacagtatactattctcagttgtatggcgtttgttgtttttagtattatatccagtaattttaggtgctggactgccattgattgggcttaatttaccttcagcaacgctgtttatattaagttttattggttgtatgatggtctgtttaactatagctactcatataagtaatctggttaacataagagaagttctaaaacagtatgcttcaattgagagagaacttgttggaacatattcaattgatgcaaaggttttggacgacatgcttgataatacaatgaaaaagtatcatcatcaaagatcattcgaccgagactataacttagcggatttgcatgctattgaagagttagttcaggaagaaagaaatggtaagtattttgataaatacctggctcatgatgacagtatcaaggatgaaattcgaatggccgttgtaccgaaacgggtagctgaggatctcttatattcagttttcaactcaaaaaccacatttggaataaccggaagaaaatactatcataaatggcatatggctcgattagatgaacagctgctaccgttcttacaagaaaaacaagaaaaaatgcataaaacaaattagattaaagtacctgaagcttttcaggtgcttttttgtttaggaaaaactttcttgtactaaaggaacgtatgttctgttaatatataatcaaaaatgtttgagggtgtgatcaagtgataaaggatcgaggtttaatgaaatgggcaacttctatgatgttgccggagcacaacgaaatgttaaagcagctgaatcttgaaatggaaaaaatgaagcgccctgaaaatgatgaacaaaaaattgaagcaatggcccttataattaatgaagcaaaacaaggaaaccaacttttaagtatctcctattttgaaaatggccatatttcatcgcttacaggctttgtaaggtcttttaagtacattgagagggaaatgttaataaaaacgaatgaagggcatattaaggctgtttcagttgatgatttgatcgaggtggagctggctgaaggagaaaagttttatgattgactatgatagccttcctaaacgtacttttttgaccgtagatatgcgtagcttttacgccagtgcatctgcagttatgctgggcctcgatcccatgaaatgttatctcgctgtggtaggcgatactgaacgatcaggaagtgttgttttagctgcatcaccggctttaaaaaaacgatttggtattaaaacaggttcgcgcctttatgaaatacctgatcatcctcaaattcacattgtaaatcctcagatgcggatgtttattaagctttccaccaatataactcatttgttttatcagtttgcttcacctgaagatatactcacctatagtgtcgactctaggggcctgcaccctagggataacagggtaatattgtgcagggcccctagaggatcattttttaatgtggtcttttattcttcaactaaagcacccattagttcaacaaacgaaaattggataaagtgggatatttttaaaatatatatttatgttacagtaatattgacttttaaaaaaggattgattctaatgaagaaagcagacaagtaagcctcctaaattcactttagataaaaatttaggaggcatatcaaatgaactttaataaaattgatttagacaattggaagagaaaagagatatttaatcattatttgaaccaacaaacgacttttagtataaccacagaaattgatattagtgttttataccgaaacataaaacaagaaggatataaattttaccctgcatttattttcttagtgacaagggtgataaactcaaatacagcttttagaactggttacaatagcgacggagagttaggttattgggataagttagagccactttatacaatttttgatggtgtatctaaaacattctctggtatttggactcctgtaaagaatgacttcaaagagttttatgatttatacctttctgatgtagagaaatataatggttcggggaaattgtttcccaaaacacctatacctgaaaatgctttttctctttctattattccatggacttcatttactgggtttaacttaaatatcaataataatagtaattaccttctacccattattacagcaggaaaattcattaataaaggtaattcaatatatttaccgctatctttacaggtacatcattctgtttgtgatggttatcatgcaggattgtttatgaactctattcaggaattgtcagataggcctaatgactggcttttataatatgagataatgccgactgtactttttacagtcggttttctaatgtcactaacctgccccgttagttgaagaaggtttttatattacagctccagatctagagtcgacgagagtataattagatttgattttttgaagagactatggggaacaccgatggatctggcgaaaagaatacaaaatgcaatctacagagattttggtgtaccagcaacagtaggaatcggcccaaatatgctaatgtcaaaactagccttagacttagaagccaagaaaagcccttcaggaattgcggaatggacatatgaagacgttcaaacaaaattatggccagttcatccattatcgaaaatgtggggcataggaaggcgaatggagaggaatctgaatcgaatgggaatcgccacagtaggacagcttgcaaattatcccttagaactattagaaaatcgatttggcatcatggggaatcagatttattatcatgcccatggtgtggatcttagcgagctgggaacgcctattaggcaagaacaaatttctttcgggaaaagccagatattgttgagggactacaatgaagaagctgaaattaaatcagtcatattagaaatgtgtgaagaagtggccagccgggctagaaaggctaaaaaggcaggcagaaccattcatttaggagtaggttatagtcaaacagtaggcggaggcggctttcatcggtctttaacaatagaccaaccaacgaatatcacgatgaaactttataaagcgtgcattgctttatttaagaaattctatcaaggtcaaacggtaaggagcttatcagttacattagggaacgtagttgatgataaccaatttcagatgtctctttttgaagaaaacagtgaaaaggaacgtcaacttggccatgttatggattctattagggaaaaatacggatcagatgcgattttaagagctatttcttatacaacagctggaactgcattaaaacgggcaaagcttgtgggtggccatcaagcataaaagtacatgaagatagtgaatgtcactattaatatttcaaattcattaaacaaaaagagcctgaagtaagtatcaggctcttttttaaaaaaacacaaaaaacaagatttctacttgaaatcttttaaaaattgtgatataatactatgtaagtaggcgtatgcctttttggttcagcttttctgtttgatgatacgggaatatcatcttcagtatctgatgtgttgattgttagtcaacaacgttacattgactataatatctcacaagtttaccgttgtcaactaggtttttgtaaaaaagtgttttgacaatagcatacatactgattatgcagatttgatggtttcaaaaagtgcatattgcctgcttaaaataaatttaaggaggtaatgcacagtgtgtaaattaacgttgcattacagaagaccacataaggttagaggacattttagaaattgtaagggaggccgtgtttggattcctgaacacgaaaggggtggaacttgggtgaatgaccattgctacccaggtttcttgcctgaacttccaagttaatactgaaggtcctcagtggcctttctgattatttcctcgctgttttggcagcttagtagctgcccccttttttaagagatatctctttagttagcaacatttaaaacttctataggatttcaattgctagacatgatatactcgttaggaagatatttactggaaacaagggaggcgggaaaatgaaaaagaaattcattggattcttggtcttagcttcttttttgttgatgtttaatacggcttcatatgcaagtggaactgacgaaaacacagagaaatcaactgctgaattgttggaaagtgtaatggatgattttggattattcagttttcaaattggccgaacagatccgacgattacaattgggatggatcaaaccaaaagtgaatcaaaacttcgtgaatacttagatgataatttgtctgaagaagcaaagaaaaagtatgaaatctatatatttaaagaggatattgataagttgaaacaagaacatcaaaagagtttacaggaataaagcagaccgactaaggtctgcttttttatatcaaaattagttataccacaaagtagcttgatttattgtaattaatttatcagtgtttccttcattttcgaatttaatgtgatagcttttccctttttttaagttccaattcatatgaaattggcctttccatccaccaggtaaagtaaccttttgggcacgacctttagccccacctctaccatcatcgtaaaatgcggatacagaaaactttctcgctgttcctttataggttacgatgagggtacttggatctttaaaagtttttccatatgtcccttttccaagccaaatgttatagtaaaaatcaaagtagcctgatgaatatgtttttttcaatacctttattggattatctgtaggctgctcttctgtaagtctaatcatgcttttcagctgttcagttgtataaggatgaatctctttgttattttcgtcaaaaattttgatttgagaagcaatctcttccttcttagcttcaatttcatcctgtgacagaattttttcctcaataggcaaagattcttttacctctgctgcctctactttgcttgttcccatgaaatcaaaaagagaaatacccaaaacagctgctattgaccagtacttgaagtttgctttcatattgaacggctcctttattcattttttaatttgctaaagttgcattgaattttcttatgttttctcactggtgaaatttttactgaggaatcctatggagtatagatacagctgataatttgagccattaaagctgtggaagctattcatggggttttgggttctttcgtaatgactcaatcagcaaaagagaaaaattaaacgataatgtgaaatctaaattagtgttgacgttggcagccagtaatttttatcaagacaaattaacccctcctttgaatgataatacaaagcaaaactaccatagagatcaggaatattacaacaaaaaacaccaaaataattgaaaattatctatatttctacaattatgtacataattatatgctttatgtacatatattctctgaacagtgaaaccagctgcagctgaagaaaagatgttgccggtaccggaaaccaggaagccaggtgcgacttgtcgtgatgtggcagctgaagaaagagatcgatgccaggcatccaggagcgaaccagctgcagctgaagaaaagatgctgccggtaccggaaaccaggaagccaggcgcggctgtgtcggtgatgcgcgcagctgaagaagatcaatgtctggaattgtgagacagaactatttggtcataaaaaagaaccagtggcttcctggttctcattgatttatggccataattggctcttatatatgtttacgtactttttgtttcctagacgtcttgttagtgctgtccacttcaaatagctcctgtctaaccattggataaacgaatttataaaataggtatccaagtgcagagcctagggtgtttaatataagatcatctacatcaaagcttctgtatgtgagtccaatcgctgatgatatagtaaactgtgaggtttctatgatgagtgaagcaataaacccagcgataataacacgctttgcttgtctcattctgttgaaaagaagaggaagaaaacatcctaatgggaacaagagtattatatttccgccgagctgatatacggttacggataaacttgagcctgttagtgcatccttcatggtgttaaaaggtatgaggttattagtttcttggaagccttctgcggctctgtcatgaattaataaagggtcagttggaattggaaatagcgtcatacaaataacgcctgtaagataaacaaaagtagcaagtatataaatacttttctctattgtatatctcggcttcttttgcacaaaaacagcaaataaacgataaacaacaaacaaaacataagcgtaaacaacgtacggaataataaaactattaagtaacactatatcaccctattcttataataagctgttacttaattgtaaatgtccccgtatcctcctgtcgatgctccattattcttctttttcataataaaataaaatttccctttagttttatttccataactgtttgtagttgaaccgttttgagagaactttttagagccaagatatttggctttgccttttttctgttttctgtatagttcaatgttaaaagtgccaccactaccacctgtgtcagcatgagtataaattttaatattactagcaccgcggctgtacgttttagaagtaacttgatgtttaaactcaaaccaaaaatcatgctttgatgcagccaatgcagctggtgccgttacagggagtagtaatgtaaaacttagagctgaagagactagaacttttttaatttttttcaagaaaaaaacctcctttaatatggtaatccaaaacaaaattaccatagggattaagcggttacaacaaaaaatatcaaaataattgaatattcactaattctctacattttatgtgcataattacatattttatgtacatatgagatgatataagtgtcaccggcttaatcttttggagaagtagcatgcagtcaccatgcctacaattttaattggttgtacatattttaaagagttacagaataacatagtaacagatgaaaactgttacgctgttacagtgttagtgggataatctcaaataagttgatgtttagttggggggagaagatgatatgaagaaaaaaacgactaaccaggtcgaagaaagaaaagtacgttcggataaaaaaacacgagttaatccttcattggatgcaaatacacatgaaaagctgaagaagttggccatttcttgtgatatgacaaagacacagttagcagctgaaattcttaagatggcgctcaacaatgagagtgtaattgactggtatcaaaaaaaatacaacaaagacgattcatatagaattatccttgcccgtattaatggtgaattgcattattcttaaccaactttcccccaggtgcggccaatttttttccagagtttaaaacaactagaacaaagtttttgattcttattatatttttcttttgacatccggaccgttttaccacaatgtttacatttcatttttatgacctccctttaatagtatcagcattgccaataaaacagattttatacagattaagtggattctaatgttgctcagggcgtctgtgttgcaactaaaaaaagtttgtcatgcaatcctcccttaaatggcataaaaaaagagcctagattaatccaggctcttaaaaatcatagtcgtattcttcttcaatagttccagtgattttttcagtgattaactgaccttcttcaatcgtttctgaagctgactttggatcagctgttttgtgttctacgtagatcgatccctgatcaattttcttcctcaaatcacgaaattctttcttcatttcttctctcatggcaattaattcatcatgaacatgacgatctttttctctattctgctgttcctctttctgttgttgcatgtccctttctatgagctgaaaggcatactctctaaaggtacccttactcttacctttactgaatgtactaatctgctctaaaacaaaatcgtacatttcatcagacatttgtgttgttcggacattaaagagtggaattcttttgtttttccccatttctaatcacctaaattgattgtgcctctttttcatttgcctgtttctttacttgttcagcgcggcttaaaacttcaaggccatataagttgagcagtcttgcatcctcagcaactatatgatttgattcagaaatatcacggccatatctctcttcagtaaccacactaattgattcttcaagcacctcgccaacaccgccaaaataaaggtatttgtaaaccttatcttttggtgcagggaacgtattttcagcttgggctattttgatttctgtgtattctttaagagattttttgatgatatcagttaaatcaaatttctgaccggtattcccgtctcttcgttccatcttagtttttccaatatttgagtatataaacttttcaagctccctaacgctatcaaagtgctctaggagtttttcttttctcaatttttctaagtgcgctaaaaacggtgcttcggtattagaaacaaaagaatcacgactttttggcggttttaatccagctggtagtaatactagatcatctgttccgccacctaaatcacaaaaaactacgtcataatttttaaattgttcggcatagtctttatcttctaggtcaaagtttttctttattgcccatcttgctacttcagattcgatcctgcacgctgcatcttccacttttatagtaagctctttttctaatcctaatgtcagcacctttacttggtgagtgcccaaaaatttagatgccatccttttctgcatttcactgaacttatccaattttttaagaagccaaattggtagcattgtttgaaagtattcaatagtaacttcattatcttcacgtttgccttttagcgcttggtaataagcagttgcagctaaaaatgttacgtatggaatatgtgactctactttattatgtaacttcttgatgtgttggttgcctaacacttctggttcagcaagttcaccaactagaaaatatctctctgtttcatcaataactgtagaaactaataaccggtcctttaaatctgccggatcttcaacgatactcgtaaattttccttcagcagcttctttagatatctctactacatttgtaggcaattcaaaaaaataaccatcaattaaattcatgtacatactgtttccaaagtccacgttcatacgagaaatattcatatttttattctctcctttgatttcactttcctcaatactagcatcttatatcactaaagtcaataaaatgaaatcacatttaaaatcagtgaatacaggctatttgaggattatataataaaaatgaaatcagtgaaatcagtagagaaaagtgatttcaggcccggggctttacgtcaaaaaaaaaatcgtgtaagataaagtcaagttaagtcaatgtgaaagttttggcattgaattctggttctagttattctaaataaacaacaaaaaaccctgttgtttgcagacaacaaggttaatagatttgatgatacatattttgtttgcgagctatttgcaaaattgaatacaaataaagaatgacaaataaaaagtgtccgatgttgcagcatcgaacacttggtttgtaagccctcacttacaatgtttaagttatgtcttcattttaccgaaaacaagtgtatacgtcaacacttttcggctatttttggacgacagaaaaccactgtttggagggtatcaaaccgtggttttctgtcgttttttgtttgtcacccagctgccgttaaggggtgtaaaataaactgacgtcaggagttgccccgtccaccgcaaacccggggatataccacaataagcgttccttgctgcgcttgtggtgaatggcgaggacggccattaacggtccggagaatgtggataaaccactaggttgcttggcgcactacggtgcgggcaactatggccaagcttctatgcagcggcacacaattgagtgtgaccgtgtgagagaacacgagacaaaccccatagaagttgcatacaggacaagcattgtatgtaaaaaggtcatggcaggcgaaagcctggcgatagcaaggcagagctggaaacctcagacgtctctatgacgctagtttcaaatcctgatcgattgcctatgtctgtccgtttttattttttgcgcgacagacataggcaatcgaaattcgccctgtttcctagaacagtcagctattctgctagtttcaagttctcaaagtcaagagaaaaacactaaataaatgcgaatttccttaaaacccagaggttttaagttcctttttaagggttgttcgtttgatagaacattagtattttaatatatttttcctgtgggatttcactaacgtatactgttattccctttggcctatcttaaaaacttgtatagattgtgtttgagccgtttagtatgatatcagtacatgcttgggttcagagcatcaaaatgagatttgaacattaagcactatgtactaaatgttc